European Patent Specification EP 3 708 173 B1, published September 13, 2023. Title: Pharmaceutical Comporision For Use In Cancer Therapy Comprising miRNA. Applicant: 3-D Matrix, Ltd. Hiroshima University. The sequence listing filed with the application follows.

SEQUENCE LISTING (32 sequences)

SEQ ID NO: 1 - RNA, 21 nt, Homo sapiens
accugaauuaccaaaagcuuu

SEQ ID NO: 2 - RNA, 22 nt, Homo sapiens
agcuuuugggaauucagguagu

SEQ ID NO: 3 - RNA, 90 nt, Homo sapiens
ccucuugagguaccugaauuaccaaaagcuuuauguauucugaaguuauugaaaauaagagcuuuugggaauucagguaguucaggagug

SEQ ID NO: 4 - DNA, 123068 bp, Homo sapiens
gtgagtggccccgggagagggaattgagggggagaaagtgggaggatgccggcgcttcctcctggagttttgctgatgttctccagtagtgttgggagtctatcaatgagggagtctagctttattcacggaggggggaaggtgttagggaggcctgtattttgtaactttttagctctttgtacgagtaatgcaagtatgcaggtttctgtcggaggagtcttttctccaaagtgaatactcgcacctttctggccagcagttggcaaagggaaattgaggaagccagagcatatgtgcgcacagaggccatctgtatctgtaaccttttcctggtactgtgggtgtgtgcggtgtactttttgtttcgggggtactctcatataggttcccgaatgagaactacttaacctgtggacccctgaaagtaaaattccttttttaaaaaacaacaacaaacctgttttgagagaggttcatttcagtacctattggtacaggagttaaccttctcagttactgggtccaatttcatgtgtgtcaggaggacactgtaacagatgtcagttactcaggaacttgagttgttaggaatcacaacttacttggggaagagcatttatcacattaatcattttataaaagttgtgattttttccctttcacccccccctttttttttttagagtaacaaattacagcacttttttatttggtttgaggctttgcttttttgaattatctttatttctgtatcaatttaggatacatctttgatatttaagtcaggaatgattttttccttccattattttaaagctgaagtttataaaacctttgacttgtattttaggtatcttgtcagagtaccaaattaaaggtttatgaaagtaattaatatttcatatacagaccttaagggttaaacatagagcagaattttatgtaagaagacatagacagtagtatactgagaattgtggtccgtctagacaactgtgggctcgttctgtctgaagccactgctgagagatactttgtgggaatgaatgtaagcctggggttatctctcttttcgaagttctccattcaggatcttgattagattaatttaaaactttctcaaacttaacaatgtttggtccttttttttaaagtaatgagttctgcaagtttattagcctgtgtattatgtgacagttcatttacatattccatacctgtgtccctaaactttcaggacacagtcagagtttgtgtttcaagaattatcaggacaagcctcagttcatcttttcttaattttatggactttcattatttctaccatcagtttctccaactgttgtcttagaataatgtctttcatttgaccacttttccctcctctggaacttctcccactgaattgtttttctttagttgccttgttatgctttggtaaggaactttaaattctgtcctttaaatgtgtactgacatgaaaatactgaatagtggatgtaatgttagaatcagagtcacgtattctgtttttcactaagatattgcaaagagaaatgtagtcattttctaaaatactgtacccaaaatacagtagaagctgtattttgggaaggaggggaggacaaactaagaaacaaactatagtttgaatgtaggttgcactctgtcaaagttgcttactaactttaggacctacttttattgcttatggattggttaaaaattacggtattttttttttttttgagacagagtcttgctctgtcacccaggctggagtgcaatggagcgatcttggctcactgcaacctccgcctcccaggttcaagcgattctcatgcctcagcctcccaaatagctgggactacaggcatgtgctaccacgcctggctaattttttttgtatttttagtagagatggggtttcaccatgtgggtcaggctggtctagaactcctgacctcaaatgatctgcccacctcggcctcccaaagtgctgggattacaggcgttgagacaccgcgtcctgccaaaaaattatggtaatgttttattgcacgtttgggtagaaatgacaaagtttttggggtccctgcctttgagatgcttttacttgtaggtggtggagacaatcaaacacaaattgcacaaagctataggagaggggggatagaccaatatttatctaagaccgcactggatgttagatattgtcaacttatagatgtgaatatatttttacatttttcactagggaaatgttgcttttggacgtgtacatatagaactaattgaagtattgaagccaaatctgggaaggtttcttttaggaagaaaagagcaagtggagacacaatatttaagacttttggaattgaaaggcataagggacagataaaattacgaagctggtttgaagggaatacagatagaggttgttgagtagtgttagggtcagttgtgtttgtgtagacacatgattacagttcaaagaagcaactgagaagagtgttcctgagagtaatttcagatgactggggagaaattacattttaggtaaaagctgtatgcctggattaggattttgtttttctagggaaccaacatttttattatatcgtggctatccagggctatacagaaggaggagtgaaaaagaagatgcttagtgtgttgaaagtggcttcttacaaaaaagagtttagaaatgggacagtagactttgctttggatgtgaaattttagggcaacaattggatactggtgcagtttcaaaacagcaaaatagtttagcaggtaatatactgaaaatgtaaagttggaattattttcaaagtatttaggtttcccagagtactgatggaaagtgaagagctgaaaagtgggtatttttagttagggggaaaatctgaatgaatgagacactacctaaaatagatgttttagaagtggataagagttgaagttaaaaaggaatgagcaggctttaaacatggccaccagtttagtcccagggtatattattctgtatttttgaaacaagctaaaatttttttttttttttaaatagggtatataggtcccttgagattaagttcagaagagtatacttaataataatttcattgttaaggaatttataaatagaaggacagatttgtttcctcaaattcatgttttaaagttcactgtgcattattatcctacgtttggtcttgatatgacgaagtgaggccaaaaatagctgacagagaaggctgcttcccttgttcacagttggtgtgtgtctttgtgtcccatacaatggaggggatatccctgtgtaggcacagtagtgctgaacatgctttttttttttttttccttttaaactttttattaaaaaaaagcaacttggcatttaaaaaaatgtagacatttttgcggcttgcatttagtattgactttaacaggattaaggattgtgaggaaggaaatatatattcacacttttttgtgttccttagttggaattctgcaccttcctagtagcttctctgacttcttaacagtgattattcaaatggcagaaactctggggaagagatgtttcaacaaggagataggtctaaggtgattctagggtgaaaatatagggattggattatatgccatatggaggccttctcttgtcatcctccactttccacaacattttttgtgcagtcgaagccatgttcagatgaattttagaaggcagccacttatagttaatgttatttactagtgaggacagtgggaagagtggtaacttcatgtactttgccttggcaacttttggattgatagggaattagagagccttgagggtatatgtttgtgtgtgtgtgtgtgttttagcacccaccagatgaccccaaaggccatgcataggctcatttcattgtactttggagatggttcttggagaagtcttctggtgcttctgacatctcattgtgtagagaaagagttggcaaactatttttgtaaagggccagttagtaaatattttaggttttacaggccacatgatctgtcacaactttcaattctgttcttatagtgtgaaagcagctgtagacaacaaggaagtgaatgaatgttgccgtgctccaattggcccataggccgaagtttttggactcctggtatagacaactgccaaatccaccaacaaacagtatgagctttattacactacaaagccaggactggctatttttggtggtctttgttttctagatgagatgtttttctctgagttcatttaaaatgattctgcataaagcacatactctactgtacaaaatacttttgccttcatggtgatgaaaactatggattgagggtcggggtgataccatctttaaagggatgcagctaaaaagtagggactacctgcatttcttatctaaagataaccacagttggcatttagtgatatactggctttgtatcatggccaaaagtatctgtaaagaagcttgtgggcatacttttgaaaccttctgaaaataaatgtaaagcatttacttcgtgtgtaaaattagaagtgtctatggttggtttgaataatatgagtcaaattataagagcattaaagtttgatactgctatctattaaagtcttaatctcttgcagtggctaattcagtgtgtagaattacacatcgcaatttttgttttgttaatttcaagtactagtgtatattaacaaatcacttaaatcatttaaatgtgtactttaaaaagctttgatgtatatacatatatatacgtatatatatatatgtacacgtatatatatacacgtgtgtgtgtgtgtgtgtgtgtgtgtgtgtgtattttttttttttttgtgacggggtctcattctgtcacccaggctggagtgctgtggtgtgatctcagctcactgcaacctccacctcctgggctcaagtcatcctcctacctcagcctctcgagtggctgggatcacaggcatgcgccaccatgcccgactaatttttttgtatttttgatagagatgggtaacaacttttggattgatagggaattagagagcctcgagggtatatgtgtgtgtgttttagcacccaccaggtaaccccaaaggccatgcatcatgttgcccaggctggtctcttaactcctgagctcaggtaatccatctacctcgacctccctcagtgctgggattgcaggcgtgagccaccacacctggccagcattgctatatttttaagagtgaatctttctcacatgtgttgttcagaaagtgtaattcactttgtgcaattttacattacagttaatattaaaatatttgtttcatatgtcagcagataccaacattggatgatggtatatttagtttcataaatcctatttattttaggattcccttgtttatggcaggggtggagattactcttgcaataatgatcactttttagttagtttgaaacctgcttttagtttatatgtagtatttctacatattgttacttaaattgaactaacaatttactttttaatttttcttcttccttttaaaaaaagagtatataatctgacaatgttagtacatcttttagaaggtcactataaagttgctttccctatttatttggaaaggattatttccttattattttaaaaaatcttttaatttttgtcttttcaagtaattttatcattgtcccaagcctaaggatgagtggcaatttaaaagacacaaggtgtgcatcttctatctgcaaatactccaaacagaaattattccagtttgttgatactttgagtggaccagggaaaaatgtgtatgtttttagtgtaactgaattgtcattacaaaaagatgagtaaagttgctgttaaataatgaattcttgctgttaatttgtcctgttcttagactttcccccattaagtataatgggggaaaatgtacacacacacacacacacacaaagtatgtatgtgtagatatacctagcgtattgtgctagatgttcatttctgcatgactgctctggaatttaggcaatattaaaagaccttacaaaatatttttaatatcacttaatatcctgttttatgtcttaatgtacttttatgtttttgctgctttctgatgatacctccttggtacttcctcatgatacctttcacagtatgtttaaatggaatgtattttctcaaagtacgtgacattttctgaacactatgggatatatatcttctagtaattatatttttacatgcaagtatctttaaaaatttcttcctattacaacttaagaattgtgaaacatttgagggagcatctgcagtttgagcacttgatctggatattggaatgacaaacttaacatttaactaaatttttctgaggtgttcttttacaatttttgagttaacacttgatttctgtaaagcagaaggcttataagaagaaaatatgagagccagtgttcgtcttgtattatcctgccatgcacgtagttgaaaatcagaaacaaacagaaatgcacaagagaccttattgcttgagtatcttctgctcttcccccatcagacctaagggacagctagtggatcagtcagatactgtgcagtttctgttgctatgctgtgtcacctttgccctttctttctatctggaagatagctactggaaatctggctgtaagaaagagatagcatgtttttttcctctctctctctgtgtgtttctgtctgtctgtgtacctgtacctagtgtattgtgttagatgttcatttctgcatgactgctctggaatttaggaaatattaaaagactacaaaatatttttaatattatttagccttttctctgagaggatcacatcctctggctttggcgttttcatctcacagcatcttaaacgaacccgtcaatgtttattatcagttccaaatgtgaagtctcaaggcaaattgttggtttgtttttggaagaatgtatgtgtgtgtgtatatatatgtgtgtgtgtgtgtgtgtgtgtgtgtgtgtgtgtgtatataatttttaaatttttaacaaaaattcctgatctagtcaatgcttatgagagtgtgtgtggtttgtataaaattattttttttagagacagggttgcttgttgtcaccaggctggagggcagtggtgtgatccttgctcactgcagccgtgaccccctgggctcaagtgatcttcccaccttagcctcctgagtagctgagtagctgggactataggtgtgtactgccacaccctgcaaatttaaaaaaaaaattctgtaaagacagggtctcactatattgcccaggctggttctcaaactccaggactcaagcagtcctcctgaaatggcctcccaaagtgttgagattacaggctggggccacagtgcccggtcagagtgtgtgtattttttaacagccttttaggattgcatgctttttaggggggtgaatgaggggtaatatacctttgcatgacattctctaggtctgagaaggagttgcttcactaaaagtgtaatttataattaccaaatggttgaaaacaggtctacctggagtcagcaacaggcagctagtttacttctcatttacgtaataaaatacattcataatatgcattcagtaattcataattcaataatttcttggcttcatggccttggacaagctatttattatccttttaattttggtggcatcacctgttgatggaggaaaacgtgtcctttacatggtggttgttaggattaaatgagataatataaagcatgcaaagctcttaatccagtgcctggcatatagcatttgacccatcagtgttaatttattaagttaaagttgttttaaagtgtgttgtagatagaagatttaaatcaggccttatattaagcccaacatttaaattcaacacttgagtttgacaaataatactgaagtaattctgtgttttcagaaacatctaaaacttcattaacattttattaaaaactgaagaaatgacagaactgttgggcttttttttaatagaaaagaaagactgatttgaacataactggaatttgaatttagtttcaaagatctcagtagtgcatggaccagaaaagaatccgtttttgaatagttagtgattatgatagtgactgtggtttaaattgcccatttagaaatagcaggatctaattcagttatcagcctttttagttgcccatctctttaacccctggaaataaaaagctttaaaaaatcattaagaagttgaacggaaattttatctgtgtcatttacatctcaaattaagatcgaaataattttgtttacatgattctattttaactacttaattttagtttttgttttttcctgaaattattagtatgtgggttttaaaaattcctttttttgtgtgcttaatatttgttaaatacaagattggttttcagaaataccttttcttcgagtagggcataatcagtgttttattggccaatacaataaataaatgcttcttgattgtttttgtatttggaaagaaattctatgttgagaacagttttggtatgctttccttcattggctgtttattgaatagaactgtatatttaaggtatatgaaaaaaatctaagctagaaaaaaagactgagatacattcttggaagaaaatacttgcaaactatgcatctgacaaaggtctattgtccaacgtctataagaacttaaatttacaagagaaaaacgaccccattaaaaagtggacaaaggacgtgaatagacacttctcagaagaagacttacatgtggccaacaagcaaagaaagctcaatattactcattagagaaacgcaaatcaaaaccacaatgagataccatctcagactattcagagtggctactataaaaagtcaaaaaataacagatgctagtgaagttgtggagaaaagggaacacttatatactgttggtgggagtgtaaattagttcaaccattgtggaaatcagtatcgcgattccttaaagagctaacagcagaactaccattccacccagcaatcccattactaatgggtatatacccagaagaatataattcattctaccataaagacacatgcacacgcgtgttccttacagcactaatcacaatagcaaagatgtggaatcaatctaaatgcccatcagtgacagattggataaagaaaatgtggtacatacacaccatgggatactgtgcagccataaaaaagaaggagatcatgtcttttgtgggagtatggatgaagctggaggctattatccgtagcacactaatgcaggaacagaaaaccaagtaccgcgtgttctcacttataagtgggagctaaatggtaagaacttatgaacaaaatgaatagacactggggtctacttgagggggagggttggaggagggagaagagcagaaaagataactattgggtactgggtttaatacctggttgttgaaataataagtacagcacaccctcgtgacatgtgtttacctatgaaacctttacatgtaccccgaaacctaaaataaaagtttaaaaaatatattctttagcactgattatcttgctagctgtgacttctccttttaaggaaagtttgctttagattttggtgtaaatgtagaaattagatgggtttatctgctagtggctctctagttagatgattaatgaatattctagtttaaaaaatttcagcattttaaatacttttctttattggtaacgatttggattatgcttctagggatctttacatttcatagtttttcaaaaaagactttataatgagttcctggatgggaagaagagcatgttctctctagtttatttgatttcttcctgattattatgtatgtaatactggaaggttgtgtaaataaatatttgggttgtaagttttcttttgcatgattggtggtctcttaattgactgctgtgtgaatttgatagtataaactagaatgcttatacagtgagtggggaagcctttttctactgagtgttatgcaggtggatttttcccccctgcggataaatactaaacttttatattaccagatttagacatttagacaggaaacaaaatttccttttttttaaaataaatgagcgggagaagagagtggggttgtacagaggtggggagagaggcagtaaaggagggaggaaagaagaggcagatatcagggagagtggctccggaagttttgagttcagtcttagtcagaggtcacaccctgttatttctttgggttgtggacatgaggtgttaccacttgttatctgtcaccctttgaaatgatgattagattattggtttttattcatagcttttcaacatttgggttctttaaaccattgaaggtttagtttgtatgggataatcagtgttattttagggtgggaaaatttccaccatacctgctaggagaaggggatggccaaagagtttttgacttacagaggagtttttttgttctgttgttttttcctcattgactctatttcgctagctttgtctgagaggggtgcttataattctatatgtgacatagtagctgagaggcaagctttggagttgatagacccaggttccagctctgctgctttgtgatttcaggcaagttatttattccatgtgtgtttcttttaaaactgggatgataataatagtacctgtttcccttatagagtaattaagaggattgagtgagataatgcatgtaagcctttagcacagtgtctgcctaagttagcatccagtaaatgttagctgctgcaataataagaaatattatagtattaagttattgttatttctgtgagggtgctggttttctgaatgctgagacattggtgatctttgctcctgaacgtgttactatttggaatactgcctttattcagcagcagattcagttcagatttactgaacacctactatgccaggaattgatctaaataagcaaaacaaaaatcctgctctcttgaaacttactttctggttaggagagacaaaatacacaaaacaaaatagatgatgtgtcactcaggaaatttggttgttggactttgtctaagctttcattaaccaaccctagcagtcttaacctttacatactttttgattgttcctgttgctgtgcttgagagtgtttggaggtaggggcaccctaaaagcgtatcatagactagctttattgtctccagcttcagcttgatcctaattttaaggcagccttaaatgatagttttcatcatttccttgacttactacttaaattggctatctcaaaactttcagtccccaaaacttgtatttcacatcattcagagagatgttgctcctccccagctgctcctcttttgctcttctatgccattttcttaagaggaggggatactagaagcatctttttagatttattttctgactagtctaactgtatacttttctttctcatattttgtgttttctaccctttatttattgttaactgatacatttaatttgcttattttctttaaaatatgtgttttttttggtctctccaattaaattgtgaaagtttttaggtcagggaccacttttctattttgaccttgagcttactctcttgaaaaaaagataataccacccagggatgttgtgagacctcaaagagataatgtgtgaaaggggtcctggagccagatccttaataaatgttagtttcttctttgaaccactctagttgctgaaactgctgtgcatataatcagtgcttaaaaaatgcttgttaatttatcttgaattgagtttgtgaactttcaattgtcacttggtggtagttttagtttttagtgctagataagattcaaaatactacttttcaagtgtcagatgataaatgctgggtcattagtggtagagctcaacagtgattaggagcaggaacttgagccatcattgtttgggttcaagtacaggctaccacacttactggttgtatgacctttggcaagttgtttaacctccctcggtttctttatctgtaaggaggggaaaatgatatctacccacctcatggttacttctttgttagtattaaacgaagtaaatgagaagctcgaaacagtgcttagtatataacaatctataacagggtccccaggggacatttggcactatttggtgatgtttctgatggtcatttgggggagtggggagagggaagggtgctactggtatctcgtgggtagaggttaggtataaacaaggtataggacagcatccacaacaaaaaaattacctggtccagaatgccagccctgccaagcaacattgggaaacccagcttagttcctttgtataaggtactttgccagttagattctgtatacatgctgattattgataaagatgagtcacagacatggataggcttcatttaacattcattttaaaagacagacatgtaagaaggttagtaggtttcatttctttttaaggttacagggaaagtactccaaaattaatctaaaagtccttacacttttttcagaaactgagaaaaggttccagatgaattttactaatttaatttttttatgacgagctattcatgtaaaagtgtattatgaatagagggcttatgagatatgagtgccgtagtgtgtattcataaagtcaaacgtacacttaaaaaacaagtatcaaggtaaatggaatgatctattgggggaaaccttggagctctctctctttccatatgttttattactcaccaagtcaagggctctttaacttaggatcttgtttttctgtgtacacttttcctgtttactgtttaaaattggacccttactaaaaatacagaaaattagctgggcatggtggcgtgcacctgtaatttcagctactggggaggctgaggtagggagaatcgcttgaaccagggagacggaggttgcagtgagctgagatcgcgccattgcactccagcctgggtgacagggcgagactcagtctcaaaaaaaaaaaaaaaaaaaaaaaaaaattggacccttaccattccttgtccatttcaggagcctcttaattgccttgcttctgttctttctctgtattcccacttgaattgactcttctttgctgggatccctttgggatcccttctagtccagatccaatctacccttcagagctccttccaccgtccccttatttctgggagagaattcagccttaataccctaaggatggaatttgaatgtactgacttttctgctatttacagggttgtgtattatctttggaagaattgggaagtcatatcattttctgtatgttgtggttcaggtgacttgtttcacttgtatccaaacactggttgtgtgtccatgtatatacagcatgtatgtactttaatgtctatttgtatgtgtgtgtacatgtatattctttcatgtatatttgtctctacaccttgctgtttcctctgcttggaatattcttttcttttcatctgggaaacatttgtctcttcagaccctacttaaatattgatctcctaggaagtgtgtcctgattaatataactagaattagttatttttttccactggttacccacagtatctctgtggcttttatagcacttaacatccttatttgtatttttcttttctactgatctctcagttctttgagggcaagagtcttgtcttagtcaacacctgctcccccaagtacctaacattcctgccacattgtagacatatagtatgttaacaaatgaatgggagagacaaaaaactggaaagcttttaaataagttctatgggggttggcaggaggggagaccacacattatcttgtcacctttgtttccaagtgcttagtgttgtgcttgcccataggtgttcagcaaatatttgttgaatgaattagaagcaaatcccaggagctgataaaattttcatgtgaacttttttcttctgcatttctagaaagcatatcctagaagtaaagtagcttagatattttggaacatcttattcttaaagtcgaccttcctatttttgactcagtagtgaaactttgatccaatggatacttcctgaatagtgcttttggctgattcctttttcacaacataggtccgttctggtgttgagtttgttggaaagatgaatatgtagtatcatttttacatcatggaggagccatcattaagtaacagtgttaaataaggactggtcccctttgcacatttgggcccaaattaagtgagtatgtactcttaagtatgggtaatgattgaggctattgaggtgtaggaaagaaagaggacaactggaggtgaagaagtgacctactagatctcttttgcttttggtaatgattgattttttttttttttttttttgagacggagtctcgctctgtcgcccaggccggactgcggactgcagtggcgcaatctcggctcactgcaagctccgcttcccgggttcacgccattctcctgcctcagcctccccagtagctgggactacaggcgcccgccaccgcgcccggctaattttttgtatttttagtagagacggggtttcaccttgttagccaggatggtctcgatctcctgacctcatgatccacccgcctcggcctcccaaagtgctgggattacaggcgtgagccaccgcgcccggccggtaatgattgattttttacccccagttatttttaaagaattggcaaggaaggagaggggtatgaatctagaagataagaatgtagattttgtaattcatgatcattattattaccatgtattgaatgtttactgtatgtcaggaactgtcctaaggatttttacaaccgttatttaacttagtcctcacagcagttcatatgaaatagctactgatgttttatggcaaaggaaacaaattcagagaaatttccaagaacacatcggaattttgacttgcagaactgggattcaaatctagatctgtcatactccatggtctatgcttttaatcatgcatgctgtctcttaagtttttattgaaaatggaaagttgtactgacataggaggggaaaatgatagaaaatcatcctattggaaggcagattaacagactcgtgaagaagcaattcccagttttatgtcattatacaaaataattgtgaaattgaagtccgtcatttgaattgatttgcattaaccctcattttttagtcttgctcttggaatcatcatcaggacaggtgtcccagatatgttagcagtagaataaatttatctaggcaaaatctgtctaagattatggagaaaactgattttatatgtgaaatgtgttgttgagtgagagttaaatcttttgaaggagattatttcaggatgagcctcaaatacattatttaggatttgaaaacctatggtttagcagaaaatctgagaatcaacatttgttagtctcttgggtataaattgcttaagtcagtgggtatctgattattctttctttctttctttatttatttatttatttatttttgagacagagtctcactctgtagcccaggctggagtgcagtggtgtgatcttggctcactgcaagctctgcctcccggattcacgccattctcctccctcagcctcctgagtagctgggactacaggcgcccaccgctacgccctgctaattttttgtatttttagtagagacggggtttcaccgtgttagccaggatggtctcgatctcctgacctcgtgatccacccaccttcacctctcaaaatgctgggattacaggcatgagccaccacgcctggcttcccttatgtaatttcttaaactatttttgtttgctgatttggtgtttgtaatttaaaaaaaatttattttttcttcttttacatactttgtagaactattccctacccagtgagtttatttatagatatttcatatttaattaatactgtgagaacatagtttttatatctgtatttttgttttttcattaggatatttaaaataatttttgtaattctgttaccttaaaaagagctaaacttagatgttggcctttaaaaatgttttgtgaaagattttctcttggttccatttaaaatactgtatttgtaactatagttaaatacatttgaactttgcccttttcagaaattttaattatatgcctttataaaattttatcaaaagttacatgcaaatactaagtatagagtgctgaagctgagcgtgatggcttatgcctataatcccagttactcgagaggctgaggcaaaaggattgctttaggccgggagttggagaccagcctgggcatcatggcaaaaccttgtctctacaaaaataaaataaattagctgggtgtggtggtgtgcacctgtagtcctagttacttgggaggctgaggtgggaggatggttttgagcgtagtagttcaagactgtagtgagccaagatcctgccactatactttagcctgggtgagagagcaagaccctgtttcaaatatataaataaataaaatagtaggctgggtgcagtggctcatggctgtaatcccagcacattgggagtccaaggcgggtggatcacttgaggccaggagttccagaccagcctggctggcatggtgaaaccctgtctctactaaaaatagaaaaattagctgggtgtggtggtgcgtgcctgtaatcccagctactctggaggctgaggcaggagaattgcttgaacccgggtggtggaggttgcattgagctgagattgcaccattgcactccagcctgggcgacacagcgagactttgtcttgaagaaaaaaagaaaaaaataagtattgagtgctgaatgatgttctataaaagattaaaaatgcctaagtggaactaaattctggtaaatagaatttaggggttggggtagaaagaatcagataagtacttcaagattttcagactttaagtctaaggctcattagtatcctctgacataatctactacaggtttcctttcttagaagtgaatgttaatatggcaccactatacaaataatatcgatatcggtatttgagtgtttattatgtgacaggcactgttctgtgtccttcatgtgtattacctcatccagtcctcacgatagctctatgaggtaagtgttgttaatatccctattttatagctgaaaatttggcatagagaagttaaacatggtcaaggtcccacctttagttaatagtggagctgggattgtttccaggcagtctggctctagagcctgggaccttaatctttattctatactgtctgtgtcatctgtaaatttatttcttatatattatttatagaacagtgcctggcacacaataagagccatagaagtactggctattttcattggcatttaattatatatgaggttggcagagcatgcattattattccatttgtttatttatactattaattagatagtagactttattcagatttctgtgtttcctttttttaaatagtcgagtttaccgaagttcttagaaactggatgattgcctccaataatgtggccatgctagatctcaaaattaacttttttaaaaaaaccacccctccaactttatttacacttccttagaaatggataaagaccaagattgggcttctgttttgatatgtcattggtttagaaaggcagaaacagcctggcacggtagctcatgcgtataatcctagcactttgggaggctgaggcgagtggatcgcttgagctcaggagttcgagaccagctggacaacatggcgaaaccatctctactgaacatacaaaaattagctgggtgtagtggcacttgcctgtagtcccagctacttgggaggctgaggcaggaggattgcttgaacccaggaggtcgaggctgcagtgagccaagatggtgctactgcagtccagcctgggtgacaaaataagaccctgtctcaaaaacaaacaaaaaaagcggaaacaaccatactaagtttacagtattgtttgtgtgcctacttggtggaagaaataaattcttagaagttacactttctttaaaaaattaaaaattaaaaactgtgcagtgttgagattagtattaccgcttatcttgctgacttgtgaaattgaattacatcacttataataatgtgaagttttagaaattgttttgatgataaagagtagcagcctttaagagaaataatataaaccatgtttcctcaaatctaaatggtcatctgtatggtattagttttccatcgctctacagaagcagtccccagcctttttggcaccagggaccatttttgtggaagacagtttttccgtggatgcggggaaggagaggcagtggggaatggtttgggatgaatcatcaggcattaggttctcttaaggagcacctaacctagatgccttgcatgcacagttcacaatagtgtttgtgctcctatgagactctaatgccacagctgatctgacaggaggcggagctcaggcgataatactccacctgcagctcacctcctgctgtgcggccgggtttctaacaggccacggaccagtaccagttgtggacccctgctctacagcaaattaacacaaatttagcagcttatcttacagtttctattggtcaggaatttgggtatggtttagctgggtctttcctcaggttctcactaggctgaaattaaggaatcagccggggctcctatctcttctgaggctctgggttctcctccaggctcaccggttgtgggaagagttcaattccttgttcttgtagatctgatgtccctgtttgcttgctggctgtcagccagggaccactttgagctccttagaggcccacccccgccaccatgttcttgccatgtggccaagttattatgttgtgtatgactaaggaagaaaaatgctggattaaaatataagacaaattcttactttatgtatgactaaggaagaaaaaatgttgaattaaaacatgatacaacacattattgcttggacagtgccttgcaaaaaaaaaaaaaaaagagagttgtggttattcttccagccacaatatctgcttcagaaatgtcaaatttattttctactgttgtgtttgtgttcttttttgtaaacaacttttttgtttcaatgctgaatcatagtattttacaggacatttaaaattaagaagtaagcgtgacttcttattgtactactaaatgtacagaatttagtaataattatggtgatataaactgccattacccaatttgcaagtgtacagggaatgacagctatgttgtgactgccatgggcaaatggtgatttgtaaagcattgttgcttttttccccccattttaagttgattttattgagatataatttatatacagtaaactacaagacatttctgtcaccctcaaaagattcctcatgccccttcacagttaaatccttccctgcaccctcgcttcaggcaatcaatgatctgcttttttattactacaaattagtttgcattttttagtattttaaacagtgaggaaaaaagaggagatggagacaggctatttttaatttttatattttcttctttgttcttagagaaatcctagtttctttattaggcattaggtttattccttcagtgtgggggtaaagtgattcttcttgaagctttctaagtatgtttcctagatgttcttgacctctgttttgcctaagataacttttctccagcatacccagagttggctctcttaaaccatacgtgcttgtgtagctccctcatccatatttctacttattgtcttttcaggaccgtaaacagaggtatttttgacttgacattctcagctcctaaataatcttatagtgttactgaggcttttcacctgtcacatacccccgtcctagtctctttttgtgttgctgtaaatacccgaggctgggtaatttatgaagagaagaggtttatttggttcatggttcctgcaggttgtataagaagcatgatgtcagaacatctgctttctggtgagggcttcaggaagcttccactcatggcagagagtgaaggggagcaggtatcacatggtgaggcaggaaaggagagaaagaggagagggggtgccaagctctttttatcagttctcatgagaacttacagaggggaaactcattcattaccttgaggatagcacaagctgtttatgtggaatctgctcctatgacccaggcacctcccactgtgccccaccctcaacattggggatcagatttcaacctgagatttggaggtgtcaaatattcaaattatatcatcccctagagaacatacctccccacccctgagaatctcagaatttcttgttgagaattcatattacagtatgagttgtaggaaacatgaaggaaagatttcccttctagtcagttcttatatttatcacttgtttcatgctccttggtgtgtatagtgttttcaggtgcaggaaatgctctgggaagaatgttgcttcttagaacgtaagagaaagggaaccccaagggaagactcaaatgaagtccttaaaaagcccacttagcttcttctgagacagcattgtccaatggaatgcaagcgagatagttaaatttaaattttctggtagctatgttaataaagcaaaaaaagaaccagccaacattaattttaataatatattttatttaacacaatatatcccaaatgttattttaacatgtaatcaatatgaaaaccatgaagactttgatatttaaaattcttattttaatactaaatctttgaaatcagtgtatattttatacttacaagacatctgaatttggacttagtcacatttcaagtaagtgctcattagttagtgactaccttagtggacagtgtagatgtagattatgaactttttaggaaaagacaatagcatgtggactccacaagaaattgtctttaacaactgtttgactctcataggttagggctttagtgtttcagaatggtttctatggttgagatgtaaagttttttatttttataaaggtaagtacatttttatacattttcattatacaagtaatgtcattgttgaagagttggaaaagtctgggtaaaagacaacaaattgtcctcacttcctcagtccagagataaccaatggtaaactttattgaatttcctctttgggaatgttgctttttaaaatcaaagagaaaatagatttcttttttgtcataattccttcctgttcacattcagacatacattattattgacaattcttttacctctttgtttaaatttatgtattctttttctcgggctgtatcctccaatagggtctctgtgagtggagtactctggagcacagtaacctgaatggtgcttccctggattagggttaacaatagaaacttcaatggcttttatgtactcattgctaaaccagtgtagttgctttctattttaactatctgcgatctctttgcatatcctgcagcttttttagttattgaggtataatttgcataccagaaaattcactctattaaatactcaattcaggccggcataatttgcataccagaaaattcacgctattaaatactcagttcaggccaggcgcaatggctcatgcctgtaatcccagtttgggaggctgaggtgagcggatcacctgaggtcaagggttcgagaccagcctggccaatatggtgaaaccccgtctctactaaaaatacaaaaattagccgagcatggtggtgtgcgcctgtagtcccagctatttgggaggccgaggcaggagaatcgctggaacctgggaggtggaggttgcggtgagccgagatggtgccatttgcactccagcctgggcaacaggagcaaaactccgtctcaaataaataaataaataaatattcggtcgttttcattgtattcacacagttgtgcagtaattatcactattaatccagaacattttcattacctcaaaagaaccctgatgctcattaaggagtcacttcccatttcctctttgcgcagtctcctggcaaccactaatctacttcctatctctatggatttgcctattttagacatttcttataaatggagtcatacagtacatggccttttgtgtttggcttctttcacgtaacacgatgttttcagtgttcttctgtgttgtagcatgcatgagaacttcattctttttaggactgaatagtattcagttgtatggagggtaccacattttattcatcagttgatggactttggggttgtttctgctttttgagatcacattcattcttcaagaacattaatttcttaatatcgtcctccattcttatcaaagctttcagtggtttcctgttgtctataaacataatagaaaaatatttagtttgcattcagtcttacaaagtgtaacttcaagttactttcttttccactcttattttccatcttgttgttgtttactgtgtctaaaatatgtgctatatatgaattataaaattatgtagacaatatagataaccttgtcatctgatctaatttttaaaaagtgaatttgaatactgccaaactaaggagtatgtgtagtatggagaatttgagaaagacaagtatcagtaaagaagaaacagtatagtaaaacaaaatttttttctgccttggtccattgaaagaaatatttagtttcatataatgtgaacaaaaaccttaattttgaatgaacatttgatacataggaactcattcaaatcattgattttctggttaactttgttagtagtttgtttttttctgagtcttttgttttaatccagatagtcagtctttttctcctttttacatgcttgaaatggtaaaaatgaaatatttttacttattcttaaaaatatttccagaatgtcttacacacacatacacttagaaacaaatacaaatatatagtgatattctctcacattttacagagaaaagcgtagtatacatactttgttttttaatttcacagtagatcttagaggtcttttaatattagcatactgagaactttctcatttttttcataatagtattgtttattccattgtgatgaatatgctattgtttttgaaactagtcccatattggtggacatttaggttgtttccaggtccactattacagataatactacagtgaataagtttgtacatgtatcatttcatatgtatgccaatatttctgcaggataatttcccaaaagtgaaattgctgaatcaaaagatatatccacctgaaatttgattacccatatttttaagcataaaggaagagataaagggaaataaatagaaaaaaaagaaactatagattttcaaaaactttgtttatagatgaaaaaatggaggattagaacttttaagtaattgtccatggtcatgcactccacagaggactgggcatggtgggattcggtggggggggcggggggctgtgtcaggatgctaacccaggtgttcctgattttaaataagctgctatccttcctgttatattcatactgcatgttatgagcaaaaggggagagaagtcgccaactttttggagaaaaagaataaaatcccagactttatttttgggatcatctgaggtgggaagatggcttgggcccaggagtttgagaccagcctgggcaacatgaagagaccccctgtctctacaaaaaaaaaaaaaaaaaattaaccgtggtgtttgaggcttcagtgagctgtgatcactgcactctagcctgggtgacagaatgagatcctagtatatgtaggtatttaatgtatatcgaaggcagcatttcagattggtgggggagaagatggattatttggtaatttatattgcagcaactttctattcatttggggaaaaagccctgtcccttgctcttactctttacataaaaaataatttaaaaatgaaagcaaaaggtaatatcgaaggatgtcgtgaggttagccttattcaatagactgacctcagtgagtactgaactcatgaaagtttcatttttttcccagtcactgtcttttgcattttccttaattgatttttaacatcaccttggattaatctcatagctttcccaatatgtttttagttatgaaaagtctatttctcctcttgccccgtattaggcttgacctgtggctggagagatctgtggtactgtttcatatgtaccgccctcctctttctctcctcccttttttacttgttctgaaaacaatgagtaaggttaaaaaattatttttcacaaacatgaaaaaggttgataatacgtaagttttgaatatgggggaaagttactctcatactgttgttgggagtatacatttttgtggcctttttggagagcagtttgacagtatttatcaaaataaagtacacaggcatcttgaatcagcagttgttcttccaaaatttagtagtacagatatactgacataactttacttgaaagaagaatcctttttataacttagtgtttattgacaagagaattagcatttagagtcatttattattctaactcttctaccaaaatggtgagatgtgttgtaatttactggacgtttaggttgttcccaatttttttgtaagtatgaaaaatgctgcagtgaacatctttgtctgtgtgctacccagtcatcactgttgagaatgtttcttaatggctatatttaggtaagtgttatttccctttatttcccctcttatactttaaggagcacaggagatctcagttttaatcgcagctcaattgcctaaatggatgtgtgacttaaaacaagctctttaaccttactgagcaggaggttctgcagatatgggcctctcagactattttatagcagtaataaatggactacctattgtcacattcttcatgatcctgtagggagtatgtgtcagtaggacaacccattgagtgacagtcctaactttcttggttcctctccctcattgtgaggtcattgtttcacaattgtatatacttactgattcaaaaaacaactccaacacttattgaggggtagtactgttcccagttgagaattactgttgtaaaaattttggcaggaattatataagattattcatgattgttatcgacttatctttattccttcatttttttttaaagcaggaagcaataatagtttacgttcgttaacctcaatatctactctaaaacatgttgtttttcttgttattaccatgaaagtctgggttaacaggagacgagactagcttcttcacagatacatacattaatttgacattatagaaaaatgagactgtatcctgacttgccagtttggttttgattggtggtttcacctttttttttagactcaggaaaacggtggcaaaaatagtataaagggtaaattctcatatgcccttcattcaagttcccaaaatttaacatcttatgcagtgacagaaaaattatcaaaatcaggagattaacattcatgtaatactgatagtctacagactttattcagatttcacccattttctcaccaatggcctttctctggtccaggatcacaatatgaaattattcacgtgttgtattttagttatcatgttttcttagttttctttaacctgaaacaattccagtctttctttgccttttgtgactgttatactttggaagagtactggtcagtaattttgtggaatattgcacaatttgtgtttgtatgttttcctatgattcaattaattttaagcatttttgattaagaatactgcaaaaatgattttatgaatcttatttagaggcacatgatgctgatttgtccagttatcagtgatactaattttcagttcctttcgttaaggtggtatcaggtttgtccactctagttgctttttttcctttgtgattcataagtagtgttgattcagattctaggttaagaaaaggaaaaaaaaaagtatcctatgggaaggtacttaaaaataagtactttgggaccaggtaattaacatttctcaccatactctaccaatttttaacttccttgctgttttttttttcttttttttttttgcagtggcacgatcatgagtcactgcaagcctcaatctcctgggctcaggtgatcctcctacctcagcctgttaagtagctgggactgcaggtgcacaccaccatgcctggctaatttttcatattgtttgtagaggcgaggtttcatcatgttgtccaggctagtctcgaactcctggactcaagccatcctgtgttggcctcccaaggtgttgggattacaagcgtgagccactgcctggccccagactttaacttttattgatgattttgtcatggtgattttctgtttccatcatttcttctgtatttacattagtggtttttggtaaggaagaactttcccttgttatgtatttatttaatgttttatgtatatcagaatggactcgcggattttttttcccctcttatatcagatggacttacagattcttctatggatttcatctattatcatcattatttattttggtgctctaattatcccaggtttggccccatgaagcctcttcaaggaggttcctggtccttttgacatgtctccatcattttgtgagggcttaactttttttttttctttttgagtcagggtcctgctgtgtcactcaggctggagtgcgcagtggtatgatcatagctcactgcaacctggatttcctgggctcaagtgatccccctgccttagcctccggagtagctaggactacaggccaggtatgtgccaccacacccagctagttttcgccttttttttttttctccaatagagacagagtcttgctgtgttgcccaagctagtcttaaactcctggcctcaagcagtcctcccaccttggtctcccaaagtgctgggattataggcatggaccaccacacctggtcagaaggcttaactttctagtagcgcaaaatgttctagtctcttcttgtgcttttctctgccccagccatgaaatcagccatttcaccaaggaatattgattccttttactggaaatcggaattcttccattccccctgcccccagtacttgtatcttaccatctttttaaaagtctttgtgtcttagaaccgtgttagatgatctggacacattaccctgatgtacagaaattagtttatacacggtaattctttttgtagcagactgtttaatttgtagcagattcattttgcactgattaatcctggaggatttcttcacaagttacattgtgtcaaatatgttatttcatgggaacacaattgaattttttccttaattttgttcggtatttgataataacaatttaaaaaacttttctaagagcttccttctaatattatatgatataggaatgtttacatttctcatttatttatttggtgtagtgatctcagaagtttttttaaaagaaaaatcttgactttgtctcaggtactctcagttcacttccatgtgggagggtcatttgccatccatccagattacctttttgattaggcttttcagtgtctataaatatttcggtcttttctgatcatttaatttctaatacatgcatatgctcctatgtataataaatagacaacttcaaatttgcagtttctagatggttggaaaagggaaacattgtggtgtgtaatttatcagccatcagatcctagatatttgagattttaactaagcaaggtattagatagaccatgttgttttggcttcacagaattcattcatattgtgcattacacaatcagtgtgcatattgcacattgattttatctgtaagttgtctttatcagtggttctcaaagtgtggtcccctgctagtatagtatcagcctcacattggaactggttagaaatgcagacttctcaggatccacctaattgcagtagttaattttaacaagcccttcggtgatcctgaaacatgttacagtttgagaaacactgctataatacgtttcatttaaattgtttcaggttgtgggggtagggaataagactaccaatttattcatcttctgtgcaatattacctgtttacctaactcttagagatattaagatattttgaagaatgtgtcccatgagattataatggaactgacaaattcctattgcttagtgatatcatagctgtcatgaagtcttagtgctgtaccttactcatgtgtttgtggtggtgatggtgtacacaaatcttctgcactgccagtcgtctgaaagtatagcacatggccgggcgcggtggctcacgcctataatcccaacactttgggaggctgaggcgggcagatcacaaggtcaggagattgagaccatcctggctaacacggtgaaaccccgtctctactaaaaatacaaaaaattagctgggtgtggtggcgggcacctgtagtcccagctactcaggaggctgaggcaggagaatgacgggaacctgggaggcagagcttgcagtgagctgagatcgtgccaccgcactcccgcctgggtgacagagcaagactccgtctcaaaaaaaaagtatagcacatacaattatgtacagtacctaatacttgataataaaggactgtgttactggttgatatatttacaatactgcactttctgttgttactttagaatgcactgtttgaactttaaaaaaataaattcactttgggaggccgaggcggacgaattgcttgaggccaggaattcgagactagcctggccaacatcgcaaaaccctgtctctactaaaaatacaaaaattagctgggtgtggtggtgcacgtctgtaatcctggctacttggaggctgaggcacgagaattgcttgaacctgggaggcagaggtagcagtgagccagtatagcgccaccacactccagtcttggtgacagagtgagactctacctcaaaaaaaaaaaaaaaattgcaaaacagcctcaagaaggcccttcaggaggtgttccagaaggcagcactgttgttgtaggagattacagttccatgtgtgtgattgcctctgaagaccttccagtgggacattatgtggagatggaagacagtgatattgatgatcctaatcctgtgtaggcttgggttattgtgtatatttgtgtcttaaaacagttttgaaagttaaaaaaattttttttaaaacaggaaaaaggcttataaaataaggatataaggaaagaaaatatttttatatagctttactatgtgttttaagctaagtgttattacaaaacaggcaaaaaattaaaacgttcataaagtaaaaacgttatagtaagctgaggttattacggaagaaagaaaaaattttaaaataaacttagtacagcctaagtgcacactgtttataaagtgtatggtagtatacaataatgtcctaggccttcatatgcatccaccccaactgactcatctagagcaccttccagtcctgctagcttaatttatgatacagatgcaccgttttacattttatataccttatttttaatataccttttatatatttagatgtgttaatatcattgtgctacagttgcatacagtattcagtacagtaacatgctgtacaggtttgtaacctgggagcaatagtttataccatggagatttgtgtaaaagcactgtgtaatattcacacaaagaagaaattgcctgacacatttctctgaatgtatctttgtcatgaggcgatgcgtgactgtataatttgagccacacatgttattttaaaaattgcaatacccttattaatgtaaaaagcagttgaattaattttaagatatttagcctgatggagccatgatattaccatttcaacataatttataaaaaaaattgttattttagattctctttgtaccaagtttttgaaatctggtagatattttatatctcaatttcaacactaactttttaccggaagtaattgatcttcctttagatttcataaagtttatggttggaaaagtagattcacatatctaaatcgtttcagacacacttaagtatttcgctacctgaattaagtaccaaaaaataatttttctgtaatatttgcatctaaattggtaaaactggttcatgttttttagtagaatgtagtagactttgaagcaaaactgtatccatttcaaaattgagctactgaagttaagcaaattcatgaactcttgtgtcaactccgtattactgacattatattcaaaaggagattggatgttaggcaaatctatattaaataaagtgtttttcaatgatttttttgtaatttttgcagccactttgcaaaacactgtcaattaaaatttatatatgttgatttatgttagaacaaagtgtaaaatcttttttattggtttgtgttatgaaaactttaaatttcaatgtaaatttataagaaagttcttataaaatttctggcataccttcttccagtttctttttattttactttttcttgtgttagcctggtcataaataaactctacctttctttggtgcttcaagttaagcttgttcataggcattgagatgtaagtgaggaaacaaaagaatactgccatttttgtcttttattacttaatagtgaaaagcatctctttctaaaatcagagttgacattagagtagatctttgtgaagttattccactatacccagtgagcaaagaacacagatgttttaaatgtattgttttttatttttttaacatttccatgaactggctaggattcatatttttggcatgtacatactgaacaattcaactctttacatagggcttttcatagtctgtttcagaaagctgaacacagatattttcaatgtgtatcatacagtggaataaaggaataggagaaacatcaatttttgcttttaaaattcctaacatagctggagctgtctgttgtgatagaaactaattgtttaatacctagctgaaattctttgacagaggtaaaggattaaaaaatatctatgccactcttgattttttttttttttttacagctacatagtgacaactttttcttaagtttagaagttctttcaaataaatttcacctaaaagatttaattggggccgggcacggtggctcatgcctgtaattccagcactttgggaggccaaggcaagtggatctcttgaggccaggagatcgagaccagcctggccaacatgacaaaaccccatctctactaaaaaatgcaaaaaattagccgggcgtggtggtgtgcatctgtaatgccagctacttggaggctgaggcaggagaatcacttgaacctgggaggtggaggttgcagtgagccgagattgcgccactgcactccagccagggcaacagagcgagactgtctcaaaaaaaaaaatttaataaggtagtgtctcttatatcacatggctcatctaaagctaaagggaaatagtaatttttcacattttgaatctgttgatttttcgtattattagaaaggtcttccatatgatggatggtgtcttaattgaatatcttccacgtgttgtaaagtatctattttagtattcctcataattttctaacaaaatttctataattgaaataatttctttaccatctctttatgtaaatgtgattttctttcttttggcgcaagaatttaagccagtttatagctgaccagagttacaagcccagatttgttaaaaagcttttaaacacgtttgttgtacatttacttctgacattgtttggctaattttgttgcttttcttctgattgtagagcagaaagttcttataaaattcactgtgtatttgttgaaaatgtctcctaatattgtctactttacttgtaaaactttaaaacccaagaaatagcttttaattttgctctgtcacagctaattgtaattgtcattcattagaaaatttctagcataccttcttccagtttctttttactttactgttctggtggtagcattagcttctgtatctctacttgattgtgtattgctgtaatgccttctttttacttttaaaaatgtgtcctcctcttgtccattcatttttaaagtaagaaaattaattatattcaaaatattaaaattaaaaaaaataaaaagtattgcgattgagttaccagttgtgatttacataggcatcactgcaacttgtgttatttgtgaaaaacgtatttaagtaaacgcagtacggtgttagattgatgagtagaaaaatactcattctaactgtaaattagttaatttttactgactagatcagtatttttatgtgtaatactagaaatgactcactgtatcctgagatgtggagtataatatgcagtacagtggtcacagtgaaatgtagtactgccaaaagaataaaactttctttagtagaaggacattttacacagcttcagcttttaaatttaaattaagtacaactaaataaagctaaaaactcaattccctggtaacactagccacatttcaagtgcttagtagtcacatgtggctaatagctaatatattagaaattaaaccttttgagagttggttatgtatgtgattaaagtattttggttacttgggactagagattacagtcatttttgatcaggctgatgtcataggaacagtaccaaggggacttctgaatcaagcaccctagaaagagctacttagaactacttgcattttctttgtggcatctcttataggcatgaaaaaatttcaaacatttttcatggataaaaggatttaatcagaaaagcatttggatatacatatttgaaatcatagcttgcctgtatgttactagagtagttggagagtggaaaagtatctatattctaaagactgtttcatcatttgggtgaaaaaccaaaaaaagagagtaattttgtttaatagctctttcacaaataaaaaaaagaatgttcatctgtagagacctatcgagatctcatcaggtttacaacaaactttagattagcaagctcaatttcagttgacatggattgtggaaagattttcagtggagctcagatatttaatatcctgaatttggatgaatatacaatttctaaaattaagtacttcaactcctctgtggttttaaaaccagtagtggccatatcttgactagttattaaagcaccaacctttttttctttattactttgcttttatcctttgagcaagttaggcaataagttctccatgtttttgatttctacagaagtaaatgaatgttattgctgatgtttatttcattctgtcttgatctcatgatatgagaatataaggagatgtctgaaaacttgttttaaaaatcctatgaagcataagttcatgaataaagaaggaagtggaacttgtcttgagagaatttgcctatttagatggtttccaaagtgcattctgctagtcactagagatggtccttgaaagagttctgtaattaagtttgaagaaacactgtgtaccataataatggcctattgaatattttaccatgcacattaatatatcaaaggctttgagatatcttacaagaaagaaacttgctaaagcttgtcttcctgcatgtcttaagcttcttccacagtgactttaagtcggacttgtctatcctgtgagaaatgctgccctctagaggcacaaattcaattgctcttaaatttgagtaccataatgctgcctgatcttagtgtgaagttgtgataattaatattaatcaaatgcatggtaacaaaaccaaatagaagaaatcttatgttgcttaattttaagaaaatatgaggaaacagaattgcaatttataaatacccactttttaaattgtacatgtgatatttttggctgctaataatcttttgaatacatttctgtatatggggaattgcggacacatagtacttcaagtctccaaactctgagtctctcctgctagcagaagccatccttccctgtgttaacaaccttgcttaagacagttaccatccatggggaagctagtttcctcataccccttcccacgatactcatgtttccatacctgtaactggagtcagactatatcatgctgcacctttgcagtcacaatgggaagaaaaggattatatgtaatttttttaaagttttttttttttttttttttttttgctgacaaagcagcaaaaccttcaggaatatgtacagaaatgggtgatgatgatgatgtgagagagaaagaaacatgcttttgcatttggctgaatgtattggtatggtgcagttatcagagattctgaattcattgttctcgttcaagtagccaggagtggttctaattgtttgctcctttggtctcagcattgacttatactaaatgaagttgaatgcctaaaaactcatagcataatatagaggaagaagtcaaaagattaaaggaaatagaactgatggagtggatttatcactgtgaccattcacttacctcccctattccctctccagtattctctactaagaggtctggaagacacttcattcaccaacctaatgagaaatactttgagggcagtgccagcatatatgaaaagtaattcaattgcttttgtctgtaggctggaggagatactttcattgaaattgtcttttttacttcagggggtgtggccagattctaggtaaggtccaggcatcattttcataaggtagcttgacaggcatgatgatcagagatgcactgacttgaattctttttggctgtgactaaatgatcatggatccctacgtctaaaatagagaggaagcctattaagatcctactttatctgtatgagcaaaaaattttaggtctcataggagaaggccttacttgaactaccataagagtgagttggccagcctgggcaacatggtgaaaccctgtctctacaaaaaacacaaaagttaacttttgtgttttgggcatggctgcgtgagcctgtggtcctggctgctcaggaggctgccccctttttgcagtttacttcatgggttatatgagaaaacaggaaggagggggatatcaccgagagattctgatattggagctgtgtgcaataactgataagtctctggttcttacctccatatgaggaacagagagagtcttgtttgtacaaggcttagttataatctgtcaggtttgaggatcttgattggaagcatagacttgatctgtatttgtggtttctcatttcaaatagcctctcaatgttggataaatttgcatgttcatgttttatagagtcagaactcaatttcctagtattccttgcagctagggcacaagcatatgacctaggctttattgatcagatgcatctgtgtaagacatgaattcagggtcagagaaatgcagggtaacagctcttgcctggaattgctttctaatgtgcatgttgagtgacaagatattgagctgtttagaggtagcagtgacagagatactagtgagccttgttgtcctaggctcagctttcatggtactagggctgaaggatgggaacaatttggtggggagacttaggtatttttcctggcatcatatctccaagtggattcttcagttctctgataattcttggaatcccctaatatattaataaatttattttctcttgaaaccacctcaaatagattctgtttatagcttagagccctgattgatcgtctaactttaaagattttatttatcgtcaaaatattttatttttctaattgagatctaaaaattgtcaagcacttatactctattttttcccttcctagagctctgcaatcctttgctgtcattttttcttaccaggaatgccaatttttgtaccttttgaattgctttttcttctttgctacttggcttgagctccactattgttatgaaacctttcttataccatcccagcagcctgatggatttttttcttcctctgaattccagtagcacttgtttagacattaagtgcaaggtgtttttttgttttgttttgtttttctgtatgcatcttagcttccgcactaaatgataagctccctgaaaactagtactatgcctctttatatcgcttgcattgtccaacagaatgtcttgcacctattagattcaaggttcagcacagtcaccctcataatatatagtgatgagagttgctgagaatcacagtgatgccaggctgaatgagctgagataataaactagttagatgcatagtctggccatgaggcccaatttccatcttcctcaaggagtctgagacttgcctctcagtagttttcgttagtaggtgatcatatcttctgaattactgtcttcttaatgttttatgagtttttttttgccttgacaaaagccttctatttctctcatgcttcctagttccttccattgtgccctctgcaatttcttttcactaagcttactatttgcagtctcttaaaatttgtgtaaattatgaaatcaaagatacaaagaaaggacagaaagtagtataacaaacacctgtgtatctaacctcagggtcaagcagatattaaccttttgcctcgtttgatttccttttaaagttcttccctccccatacttttctcccttctttggaggtactcattatcctaaagtccttacgattatttccctgctgtttttgtacacataaaacatttacacaaaagatgacctgtgtttttttctagatgtgttcatattgacatgtgtagatttagttcattcattgtaactactgtttagttttccaggttgaataatgctaagttttatagagataatgcagttctaccttttggcaaataatattgtaatgctcgtacataggtacttactgtaattttatctaggatagatacctgaaagtagaattgctgaatcacagggttcaggtgccactttatcaagtattgccgagtccagtccaaagtggagctaccattttatacccattaacatgtttccacacttttttttatcaacatttaattttatctagctatgatttttttgcctatttgaaagatgagaaatggagtttgatgattttcattttcattactttgatttatagtaaagttgaatgtctttgcatagtttttgatcattctagtttcctattctgtgaatcttttatgttctttgctgatttttttcctattgggtattgaaccttaaattgatttgtggtgattctttttataatctggatattaatggttttggtaatatgcattgcaagtatctcatagtgtgtgtgtgtgtgtgtgtgtgtgtgtgtgtggtttttttttttttttttttttgagatggagtctcactctgtctcccaggctggagtgcagtggtgcgatcttggctcacacaaattctgcctcccgggttcaagtgattctcctgtctcagcctcctgagtagctgggattataggtgcccgccaccacacctggctaatttttgtatttttagtagagatgggatttcactgtgttgtccaggctggtctccaactcctgacctcgggtgatctgcccgccttggcctcccagagtgttgggatgacaggcgtgagccattgtgcccggccttcgtgtcggtttttaacattgtttaaaagtttcagatttactacatgagttcatttgtagaatctctcttctgtatcatagcttctttggtctgctttcatgtctttacaatattgtgttaattttaatagttttgatataaatcttgttatctgataaggtgaatcttctctcaatgaaaattttgggtcagctaatcatatttcaccctgaccctaatgaaaatttaacagaaaacaaaccctgttggaaatgtgattggaatctcattgaatttacaggttacagtggggatagttgtcacctttacattggttgactgtcattgatatttctgttcaatacagttctatttttttcttttttctttttcttttttttttgagatggagtcttgcttttgttgtgatctcggctcactgcaacctccgcctccctgtttcgagtgattttgctgcgtcagcctccccagtagctgggattacaggcgcctgccaccatgcctggctgatttttgtatttttagtagagacagggtttcgccatgttggccatcctgaccttaggtgatctacccacctcagcttctcgaagtgctgggattataggcgtgagccactgcgcctggcccagttccatttttttcttgatagaagtcttcattagattttttttttttaggtttttatgatttttgttaccatcgtgaatggcaaatttttataaaaatactttttgttactggtagctacaaaccaattagtataagagacaaattgctaagaagcaagttgctgtttgtatcttgattttgtatctctcaatcttgctgaattcttagttgtttttgtttgtttgtttgaggtggtgtgtcttactctgacacctaggctggagtgcagtggtgtggtcactgctcaccacagccttgactgcctgggttcaagcaattctcccacctcagcttcccaagtagctgggaccacaggtgcatgtcaccacacccaaccaattttaaaattatttgtagagatgaggtcttgctatgttgcccaggctgctctcgaactcctgggattaagcgatcctcttgccttggcttcccagagtgctgagattacaggcatgagccattgcacctggcctaaactcttacttctaatgatagattctcttggatacctcatgcagataatcatataagtagtgaataaagatggtttttgttgctttctaagcctatgtctttatatttttcttctgttattgacctatgtaggaccactttactaaaattgcagcttttcctgggccttggctttatgtgtgtgttaatgtatggagtagaaaggggtatctcagaactgaagtctcccactaagggccaaaagtctcatttctagtccctacatatgagtcaaaggataaatataggttaagactagcaacccattgtagggaagaaacattgccaacttgtagcctaatatatatatttttaatatgttactgttttttccatgttactggcacacacttaaagatttctgtttcatggtggctaaaggattaatttaaaataattttttttttcctttttgagttgagtttcactctgttgcccaggctgaagtggagtggggtgatctcagctcactgcaacctctgtctcccggtttcaagcgattcttctgcctcagcctcctgagtagttgggactacaggtgtgtgccaccatacccagctaatttgtttttttttaaatttttagtagagacggggtttcaccatgtaggacagggtgatctcgaactcctgacctcaggtgatctgcctgtcttggcctcccaaagtgctaggattacagacgtgagtcaccacacccagcctaaaagaattattttgatatatcctttctgcatgaaatttctgtgggaaggcttttcaggtgatctgatctgatacagtgttaggactggaagtatagcttatactatataaatttccttaattgaaatttcacattatttaggaactctgtaccctgaagctgtctcactctggtatttaatgtcctacaattagtttaagagagcaagcttgggtaagtttcttaaaacttccttatatttgtttcttcatcaatattagtagtatagtatcatctcctatcttatagattattataagaaataagttaataatgtaaagcatttagaacagtattagttattggtctcaacctccttttagctgttatctacagcctttctggtagattttacttattctgggaagatagtggtgtattcctcataatctccttgtacattccaggtcctacaataattctcaaacattttagcatccttacatagactctccaatatcctggtcttatttccctgatctcctcaaatctactgatttttctcttcctcagacaagtgatttttcacttatttggtaaaatcctaattctggattaactcggttatcagattctttcattcctataccacctgaatgctgcagtaaaaagttacctcaaaggacatttaaaaaaaattataaattcatgattgttgatcacagaccctaatactgcatgggaatccactgcattatccttgtcagctagtttcctcatctttaccatgactgtttcaatcatctgttctcctcagacctccaacatgccctttctctttctacagaaaacttttcctgttactttccagtgaaaaccggagtacttggtgcaacccttagttgcccactatcttttctatattttctttcttcttaatgttaaaatagaggtagtcttgctttctatctaaggctttctccctttctctgcagtaccttatgctgttgatgatttcccttttttttgtatgtttaacttttctttacacttgattcttctcgtcagtatttaaacacgcttaattcctgctattaaaaaaataaaaacaataagcattaatgggtaccacattactgacctttctgttctctttcctagccaaatgctagaaattattgtttccatttctcacctttgactcacctgtttagtttattcattccactgtaatagtatttgcttatgataccaacaacctctctgttagtaaattaagtgaatatttttaaacttggtcttatttgatctctcacttggtgtgctagggcttctataaaataccacagactgggtggcttaaacaacagaaattaattttctcactatgtggaggctggatgtcaaagatcaaggtgttggcaggtttgttttcttctgaggcctctctccttggcttgcagagggtgccttcttgctgtgtcctcacttggtttttcctctgtttgcatgcatttctggtgtctgtgtccagattggattagggcctggaagatgaatttactcacctctctaaaggccctatatccaaatacagtcgtgttctgacgtactgggggttagggcttcaacacgtgaattttgggggagacagtttggcacataatctcctagcaggtttaaacagttttgaaaaactatccttggctggacgcattggcttacacctgtaatcccaacactttgggaggccgaggcgggtggatcacctgaggtcaggagttcgagaccagcctgaccaacatggtgaaaccctgtctctgctaaagatacaaaaataagccaggtttggtggcacatgtctgtaatcgcagctactcgggaggctgaggcacgagaatcgcttgaacctgggaggcagagtttgcagtgagccaagattgcgccactgcactccagcctgggcaacaaagcgagagtctgtctctggaaaaaaaaacaaaaaacaaaaaaactatcctttaaactctttggttttcattttgcctctctgatctattgctcttcagcctttttttaacaggcttctcttctgcttggttattaaaagtagaaatttcttgagtcttggtcctttggtattttctgcttctcttacttctgttatttctccccaggcagtcttaccactttgatttccatttatgaaggaactgcatacctgttgttccagcacttaatttgcctgagtttcagacctatttaataatgccatttagcttatcctagaggtaccttaaaaaaacgagttcaaatctgaactcataataatccccatccatgtgatttgaccctaatctacctccttagccttactattctttgttactctttgccatagctgcactatagcaaagcacggcctcttggtccaggcgtaatataccttttcctccagagtctttgctcttatttcctatgttaatatgctcctcatttttcatttacaacattacccagttttcaatacatacaaaagataaaaacattagttattagggaaatgcagacttaaaccataaaataatcactaaaaccaactagaaggggtaaaattaaaaagactgtcaactacaaatattctaggaagccatccagaacactcgtaaattgctggtgtgagtataaaatgggagagccactttggaataccactggcaatttcttataaatttaagcatacacctttggatccagcaattctacttctaggtgttttcggaaaaggaatgaaaacatgtccacaaaaaacttttaaaaattatatttacagtcgatttactccttacagctgacaactagaagcagcccaaatgtcaataggattaatgactaaaaattttttggtatattcatacaatggaatgccactcagtaataaaagaactacagaatggcaaatgtacacaacatgacatggatgaatctgacatacttggcaaaggaagctggacatgatactgtattattccatttatattaagttctagaagaggcaaagctactctggagtgaaaaaataaaaacagaacaaaggttgccttttgcttctggaaaatggtgatattcaactgggagggtgcataaggggccttcttgaagtgatgaaaatgttccatatctcatagaggtgtgtgttacatgggcttatctattaaagttgtacagctaagaagtatgtatttcaatggcatacatgtatcttagataaaataaacaagttttatctaaaaattatagaaataattgagttaggtgacagggagtgggaggtgtagatgaaagaagaattgcagaacgttggtggttgctgaagttgagtaatggatgtggggaagtttagtatactattttgtttgttttttgtgtgttcaaagttttccatataaagatctttttaaatcaaagttacgaagacacttaaacagcacctgtggtctgactgccagcttaataaagaatgcttactaatgtaattttcttctctgtgaatcgtaccctgattcagcactcctttctccccaccagccactatcctgaattcctcttgactttttaagacatcttccaaatatcattctaaacgtcacgtccatgggggaaagccttttctgattcagaacactcactagttttaagtgcccctgttaagtcctttcatagcttttatcttaattatgatttatttgcttaactattatcaacctctacactagactaagcctaagtttttggagggaaagatatatctattcttgctgttttaatgtctagaataataatacatttattgaatgattatgttggtgtagttttttaaaaaaattgaaggatacccaaattgaagagctattctattactgcttatgttgtaaggtcagtatgttataaaatgtatgaatgtgagagaatgactgagaaatgataatggtttctttctgattttattggcatctgataaaaacaaggggcaataaaactgtgttattagatctggaactatatccggaaagtcctgtcagttggttctcaaatgcccttgagctttattatgcttcttccttattaatgtattaagccgtgtgagtgaaagacccctttcctctttacaaagaatattctaaatcacctcttttttctctcttctctaatgtgcttcttcctttgactattagttttggtatttatcagggacagcgatctttaagagcttgttgttttgttattttttgtactgcttgctgtatgttttaaattttgatatatcttactgccaaatgaaggtgtgagctcataagtaataaagatagaaaaaatctgctttgcttataattataccattaaacatgttgtccttaatgcagatacacactattggtattgtaggtgcaggattatgttttgatttttgccagttcatatttccatggagtatttaggcaattttaacaacatagatttctgtaatgaatgtttttttaacttatgctgctgcttgagagacagagtcagactgccagggtttgagtcctatgcccaatatttcctagctctgtgacttttgagttatctgctttttgcctgtttcttcctcattaaaacagagatactaagtgtaccttatagtgttgttgggagggctatttgaggtagtatatgtaatgcctggtacttattaaatgttagatcttttttactttcttgggttctagggagtccaataagtaacaaatttttcctctaaggtttttttctttattggtggcaaaatatacatagtataaaatttacatttcaaccatttttaaatatacaattcagtggcatcaagtacattcacaatattttgcaaccatccatctctgtccatttccagaagtttttcatcatcgcaaataaaaacttgatacccattaaacaataactcccatctttcctcccctgatttcctggtaacgtatgttatactctgtctttatgattatgactattctaggtacctcataaatagaatcatacagtgtttgtcttattgtcctctcatttcatttggcataatattttcaaagttaattcatgttgtagcgacttctagttccattttttgtggttgaagaaagtacttccctaatagaaatgaaaacatgtttgcaaggctttttttaaagaatgcttatggatttagtcataataggtaacaactgaaaacattggtatggctgggtcaagttggactaattcactgtagcccagggtcatgtaagaacatggagttttcaaggtaggcatgggggtggtattgaggggagggtagtaagcataaaagacagtgctcagaagaagataagggtgccaggtttcagttccagggatgttcacagtaaggattacagtgggctaaattttaagattaattttataaattctaaacacatcctgttgactttaactgcaactcttaaaatgtatcaataacatgactttataattcctggaaactgatattttcccaatactttgaagaggtttaaaaatagttgactaatattagaaccaatatttcatgtattgatttttctctttaagtgacagttagtttagaaaatgctaaacttaagttagcagtatagagtaggtatatagttatactgagtatgaatgtcttggtaggcttggaagcctaccatttatgtcctcttgaggtacctgaattaccaaaagctttatgtattctgaagttattgaaaataagagcttttgggaattcaggtagttcaggagtgacttttctaaaaaacagaactgagcaccatacactacttcttatagccttttaattactgccaattgcctagaataaagttcaaattcgagggcaacacaaacatggccctttgtgaactgacagacatttcctaataattccttacatacatgatacccttgagccttacagaattaagaatttctgaatttaccttggtgtttgatgcatctgtgtttctatacgtgctgtttatttacctaaaatagactattctctatttagcctcaaaagtctcatggaaggttttaaaaaatcctgtctaagctctgttaattatattctttatactattatatttagtagttaatattataaactaccttacagtaatttttacagatacctggcttactccctaaattgagttgcttgagggcaggaattgtgtattaatctttgctgtattttctttgccttgcttactgtagttgattggtgctaattgaataaatgaacatttatgcttttctttttgagaatattatatgggtagttcctttagttgtttaatagaagatagcacagacttctatacagattggtttttatgggaaaacacaagagaataattaattaaaacataatttcatctagaaatttctgcagttggagcgaatattttttaagttattaacttacctagagtggaagattgaatttttgaatgatagtgttttagttattaaagtaaatggcatgtaagagaacttttaagttcatgtggcaaaacagggaaaaattgcaaagttagagtctgtaaggtttctgatgtttcatagactaacaaaaggttgctttattagcagcattaatgaacgaatcgctttattggcctaggcatactggtagcattgtcgttccaaagagctgagagttcttatttcaattcatgattatgttagacaagtgaagtgaaagccgttgaccttctcttaaggagaaaatagaaagtttttacaaatagattatagattaaagccttttaaggaacatgatgaagaactaaattactgctaaatcacttgaaaaatttatatttttttatgcaccagtcttataacagtaggttttttatagacctattaattgatatttaaaataataactttaataggatgattttgtagagttagtcaaagtgattgacaaaagcaaattattaaaatagtcaaactttcaattctccaaagaatgttcagttttaaaagcaatatgagatacaggaagtattaaactggagatgtaatgccacttggatggcatacttttaacattattttttatttgtttaaatggaatgcattttgcttattagaatcattttggaagtgccaatttgcttctgttaatttacattaaagattaaaataggaaccactggtgaccttctaaatcaaagttcttcaaaacggttgttttaaacagcaagaattacagaactaagtattgtatagctattaaaactgaaaattatgtagcagcagtccattttaaatttaacaattttaaatgatacttcaaaatataaaaaatacaaggaagaatataagatgcttatgtatctgtactgccaaaatttaacaaatgttaactttttgctatcactgtttcagaactttttaaaataaattaaaaatataattgaagattactaatctcattcttttgcctctcttctcagaggtaattacttttctaaaggtatcctgtaagttttcaatactttttaccacatatttgtataaaaagataaacagtactgatttccttttaaaatgtgaataataatatactgttggcataactttttaacttgcttttttcactcagtgtttatttacatcaagatttattcatgttgatatttgtatgtacttaaagtttgtttattttatcctctgaattattagtttggtccattatttatgatgtttagtttgattacttggttaaggtggtgtgacctgatttctctattgtaaaagtatccttttccccttgataattaatcattaatctgtggggtaatgccttgagactgagtaaacattgtttctcaacagcctttcacccagtgtttttaacatccattattgatttatgcctgaattattggttacattgatgcttgcaaaatgattttctacatctattattctttccacatttattagctggcattcttctttctgtaaaggagtttctgtcctttcactaagggctcatggtttcttcattaattcggtgaactaaaatccattattgttatgtagtcatgcactgcatatacgacattgatcccatgagattataatggagctgaaaaatttctatcgcatagtgacgttgtagctgttataacatgttaggactaacgtcacaaccaacatattacatgtttgtagtgatgttagtgtaagtcaaatctactgtgctgccagtctaaaagtatagcacatataattgtgtacagtacataatacttgataataataataaacagctatgttaacggtttatgtatttactatgctatactttttgttgttattttgaatgtacttctacttattaaaaaaaaaagttaactgcaaaacagcctcaggcagttccttcaggacgtactccagagacattgttattataggagatgacagctctgtgcatgttattgtccctgaagaccttccagtgagacagtatgtggaggtggaagacagtgatactgatgatcctgaccctgtgtagggctagtctaatgtgtttgtttgtgtcttaggttttagcaaaacagttttaaaagtaaaacaggaattttttaaaatagaaaaggcttgtaaaataaagataaaaggaaagaaaatatttttgtgcagctgtacaatatgttagttttacgctaaatgttattacaaaagtcagaaaagtttaaaaactaaaaagtttatatgagctaaggtttattattgaagaaagaaaatgtttaaaaatagatgtagtgtggtttgagtgtatatttacaaagcctacagccgtgtgcagtaacgacctaggccttcacattcactcttcactcaatcattaactcacccagagcagcttccagtcctgtaagctccattcatagtaagtgccctatataggcatatgattttaaaaaatcttttatactgtatttttactgtaccttttctatgtctagatattctcagacgcaccatgttacagttaccaggcagtattcagtacagtaatatggtatacaggtttgtagcctaggagcaatgggctataccgtgtaggcttgtgtaaatacactctgtgatgttagcacagtgagggaatagcctaacaaacacatttctcagaagatatccctgtggttatgtgacgcatgactgtgtatcctttggtgactcaaattgttaaaatttagccagcgagaactcaatcagtctggtttctgtttctttgacatgccccctcatttttatagcaccagtttgctttgtggcacaacaaaacattctctccttaccttatggttttcttaccccagacctggacttggctattttaccaaaagttcttgtttctcttagtggggaatggtatttggaagccaacatcatggatgcattactgggtgtcattgcttctattggttcttttcattagacagaataagaaaatatacttttaaaaactagtgatatttgaattcctagtgacaccaaggttcttttctttccttgtttcatattcctcttccataatgaagatccagtttaccaataacatcaatatatgtttattcatttgctctgtcttatacatgatataacattggaattactatagcaataccactactaataataatctcaataaagtttaagatttctatgcagttttttatttatagcgtatagcccagtgaaggtatatagtcagatcgctatgcttatagttattttaattatatttttcacataggcaatttgaaactttttctaataggaaggttaagcctatttacttatcttgacataactagtatgtttaatctaactgatatgttgtatttactgttgttttatgttatatatgtttttcttttactcttttttaaaaagttatttttactaatacaaaaatcttcctttctctagatatttagaatgttggtcttagctcttatagtttcccagtctttttggtatttttgttgtcattactatgtttaattttgttaactagaattcatgttttcttttcttcatccatttaattgggctttatactttttttttttttttttgagacagagtctcgctctgtcacccacactagagtgcagtggcgcgatctcagctcactgcagcttctgtctcccaggttcaagtgattctcctgcctcagcttcccaagtagctgggattacaggtgcttgccaccatggctggttaatttttgtatttttagtagagacagggtttcgccatgttggccaggctggtctcgaactcctgacctcaggtgatccacccaccttggcctcccaaagtgctgggattacaggcatgagctaccgtacccattctatatattcctttgcataaatgttgtgttctgaggaaaatttgtgtctgagcatttaataatttaaaaaattaccatgtgagtggatttattttatatgaataatgtgccacatgtaagttgttctgcagttgattttccctttttgtggagcttttacaatattgttagtatgtttacttgtccctttttccccttgtatgtgtagccaagtaattataaaaaatggtgcactttgccatatctgagcttctctttttcccctcaagtagatactgtgcatttgaactgcaaaaagggtcatattcttgctttatctataatctcttttaaaggcaaaggctgatggttactttttctttaataagaatcttgatttttcattttgtatatttgatatttatcattttaagaaaaaaaaatcctctatacatagttgttagaaatttatgtagaatggatgttggaacccaatcataaggctgtaaaaccataaaataagtagtaataaattttaaaaaatgaataggatttgtatgaagaaaataacaacacttcattctaggatcaaacaaatgaagagagagctatttttcagaatgaaaaaccaaatagtgttgcatgtagactctattcaaagttctagtctgtaaaattaatagcaattctagtcaaaatagctgttttatcttttgagaagttcgggaagtttgacaatctgattgtcaaatatatgttgtagagtatgttaatgaaactatccagtgtaaaatttaaaaataaagaccagtattgttatattgtactgtattgcttgctatactgtagtggtgtagtaattaaaacaccattctagtgatacaggaatagggtccaaataaataaaaactgagaaggaaattgtatacacatgcaagtgtgtgtgtgcacacacacacacaacacagaaagggtttttttttgttttttgtttttgttttttggagacagggtctcactttgttgcccaggctggagtgcagtggcatgatcatggctcattgcagccttgacctcccaggctcaagcaatcttcccaccttagccttgtgagtagctgggactatgtgtgccactgtttccaactaatttttgtactttttgtagagactgggtttttcatgttccctaggctggtcttggactcctgggctcaagtgatccttcacctcagcctcccaaagagctgggattacaggtgttagccaccacgcccagcctcaaaaagctttttttttttttccctataaagagccatatatctaaaaagggaaacagatttgactctattacaatggaattctgtgagagaaaacattttaacaagatcagactatctagtagaaaaatatttgtaacatatagcaaagttttaacaaacataataaagaccttctaaaaattaataaaattgaaaaaatgggttatgaataagtacaaataattcaaagagtgtacacaaattagttttcatagaaatatgcataaagatatatgtacaagtatgttaattttagcattatttataataccaaataataatattccaacaaaatagttggaataatctgaatgttcaccagtagggaaatggtacatctgtattttagaatattagcaagctgattaaaaagaataagatctttgtgaccaggtatggcaaaatatcccacattattcatgaaactatagaatgatctgtgtagtatgatctcatttacttagctcagtaggtctattgtttgtggtaaacttaaaattattttatttatcttataggatagggacttttaagttaacctattaatattattaggaactaaaatatatcactgtaagagaataaagacaaatatagaataaaaggaactaagaaaaatattttacatcagattaattggaaatattggtatgaatccatgagtaaataaagaaatatctctccccccaccctgttctgtctaccagaaaatataagaagcatggacaatctcagtagcaatggttacatgcatcttggttgctaaatatggctccccattgaaagaattcaagatgtcttagaaaaatagatgatcccagttcttaggaaaacacacagcaagccagaaaacaaggaagtggtgaaaaactgaggaattatgtaaaaaagaaccaactcaaaggagttctagtggccacctccgaaataatgattgcaatcacaggcatatcttggagatgttgtggattcggttccagaccatcacaataaaacaaatattacaataaagtgagtcacacacatttttgttttcctagtgcatataagttatgtttatacaatattgtagtctgttaagtgtgtaataacatgtttaaaaaatgtacatgccttagtttagaaatactttattgctaaaaattgctaataatgatcaactgagtttttagtgagttgttctaatctttttcctgctggagggtcttgactcgatgttgatgactgctcgccagtcagggtgatagttgctgaaggttggggtggctgtgacaatttttaaaaataagacagcaatgaagtttgttacatcaattattctttgatgaaatatttctctgtagaatgtgatgttgtttaatagtgttttacccacagtagaaattcttcaaaattggagggcagttctctcaaaccctgctgctgctttgtcaactaagtatgtaatattgtaaatcctttgttattatttcaatgatgttcacagcatcttcaccaaaagtggattccatctaaagaaatcactttctttgctcttttttataagaagcaacacctcagccattaaaattttattttgagatttcagcaattcaatcatgttatcaggctctgcttctagttctcttgctatttctatcacatctgcagtgatttcctccactgaagtcttgagctcctcacatccatgagggttgggatcaacttcttccagagttctgttaatgctggtgttttgatctccactcatgaataatgaatgtttttgaaggcgtccagattgatgaatccttcccagaaggctttcaatttactttgcccacatctatcagaggaattcctatctatgacagctatacctttatgaaatatatttcttaaataataagatttgaaagtcaaaagggcttctcaatccatggcctgctgaatggatgtggtggtagcaggcatgaaaacaacatgagtcttctggtatatctccatcagagctcttgggtgaccaggtgcaatgagcaatgtcagtgagcaatgagtagtattttgaacggaatcttttattctgagctacagtctcaacagtggacttaaaatattcggcaaaccatgttgttaaatagatgtgctttcatcaaggctctgttctgtttgtactgcacaagccagagtagatttagcttatttcttaagggccctacaatttttggaatgataagtgatcattgttccacttggaagtcaccagtagcattggctcctaacatgctgagtcagcctatcctttgaagtttggaagccaggtattgacttatcgtttctagctaggaaagtactacatggcttcttcttccagtagagagttatttcatctcaattgaaaatctgttgtttagtgtagccaccttcatcagtgatcttagttagatcttctagataacttgctgtaacttctccatcagcacttgctgcttcatcttgtacttttatggagacagcttctttccttaaacctcatgaaataacctctgctagcttcaaacttttcttctgaagcttcttcacctctctcagccttcatagaattgaagagaggactttgcactgaattaggctttggcttaagggaatattgtggctggtttgatcttctgtgcagaacaccaaacctttgtccatattagcagtaaggctctttcttgttcctattattcatgtgttcactggagtagcacatttaatttccttcaagaacttttcttttccttttttaacttggttaactggcacaagaatcctagcttttggcctatcttggccttcatcattccttcctcactaagcttaattatttccaacttttgatttaaagtgagtaatgtgtgactcttcttttcactccaacacttagaggccattgtggggttattaattggacaaatttcaatgttgttttgtcttagggaatagggaggtctgaggagagggagagagatagggattggctggtggttggagcagtcagaacacatgcaacatttatcagttaagcttgccatcttctgtgtttgtgatttgtggtggcccaaagcagttaaaatagtaacatcaaagatcacagatcaccataacagatacaataataatgataaagtttgaaatattgtgagaattactaaaatgtgatactgagacacaaagtgagcacatgctatttgaaaaattgcaccaaatagacttgcccaatgcagggttgcacaaaccattattttgtaaaatccacaatatgtttgaagtccaataaaatgaaatgcagtacaaggaggtatacctataattgtaaaacctttgattgaaaaaaataatccatgagtccagagagataagaagaaaaggaaggccctcctttagagaattgtagtagcagtgttagaactggaaaactgtactgtaaactccaaagaaacaatctgtgccaacagcatcaatggatgccaaaacctttaggtgtaagagtgctgtgaacatgatacgtatgcagtggtgcccaattattctgtaaatcttgtacgactacaaagggaaaatgtgcctttgcaatagatctatagattgccacttgaactaagtggtcacacttataatgggacagcctgataccatgttccttttgttatgatataatgcggaatgatgtaaccttgggtgtattcttgcctaatgtttatctacaatccagtcaggtttctagacttgatcttgtttccaagaaatacaggaagttgtggagtaagtcagaatacattctgggaagcagtcagacaaatctaggatgtgggacattctgtaagaaaactggccatgagtcctgacacatcattgtcttaagaaaaagatatgtgtgtgtgcgagagactattctaggacaggcgagaccaaagagatttaacaggcaaatgttatacataaattttcatttgcccttggattgctctctcaaccctgaaggcttaaaaatagatatctttgagacacttgagaaaacatcaagatactagcttaccttatttttacttttttttgactagatgtcttaatggttttattactttgtaagacttgttttaaaagatatgtttcactactcagtatagtctatgataaaatcagtaaatataaaatatttgtcatttgcatctcttaggaggttcgtctccattgatgaaagctcagcttatgtgtaactgtcttccaaagtagcttgcttggaaggacattcactatcatcatattctgctttatttcatagctgtgtaatcacatctactacatccttgtttatcgtttattagattactgcttttaagcctattttagttctttaatctgagaataacagttgactcagttaatttcattaaagcaagattgcctgtaatttttttataaccttagaaaagtactatgcccaacagcaaaacaaaaacctaattcaaaaatgggtaaaggacttgaacagatatttctccaaagaagatataaaatggccaataaacacatatgaagagtctcaacaccagtagtcattagagaaatgcaaatcaaaaccacatttagatacaatttggctattagcaaagacacagaaaatagcaaggattgggaaggatgtggagaaaattggaaccatgcctgcactactggtgggaacgtaaaatggtacagctgctatgaaagacagtttaccagttcttcaaaaagtttgatgtagaatgattgtatcatccaacaatttcactgttaggcttatctccaaaagaattgaaagaagggacacaaactggataacttatacagcagtgttcatagcagcattactcatactaaataaaagatgaaaaaggccaaatgtctgtgaacagatgaatggacaaatgtgtttatacatatagtagaatattattcagccataaatacaaatgaaattttggtacatggtacaacatagataaaccttgaaaacattgtgctaagtgaaataagctagacagaaaatattgtatgattctacttagatgagataccccaagctggcaaatatataaagctggcaagtataatagaagttactaaggcctagggtgagggaggaatgagaagtttgcttaatgagtatagagtttctatttggaatgatgaaaagttctggaaatgaatagtggtgataattgtacaacattctgaatgtactcaatgctactgaattgtccatttaaaaatggctaaaatagtacattttatgtatattttatgatacaaaaatatttttaaagtaaaagtttgtattttgatgttacttgtgaaaaatattttcactaataaaattttgttgtttcattgctgcctctttgaaaatgtattaaaaattatatgcattttgaaatattacagctatataaatgaaaaagagtatcagtaaagaattttagctcaatactctcatatcatgttatttattgtcctttctgtttcacattaagatatacagagtcaacaatttaaatttgcagattaaaaaacactttctgcttttggccctatagaaataaaccaaactggaaaaggtgtcatgtttcctagattgtggacacagaaaaagaagagctcaaaaggacaagtaactcagcacagtagatggttattgacctgatcatatttaagaatatcctaaaaatgcaaaaatgttaagaagcaaaactgggaaatactgggatgatatatgaaaaattcaaatgacaaatatgcagtggttgagtatttatgggtttttttggggtttactattttttcccccaaatttaatgtctcctcttttaaatacttctaccggattctctttagatgatgctgcaattggattgagacattttcattgtttggctttgtaagatttccaaatgcgtatagttgttaaaatacgtattcaatgagggtggaaggaaacacacaaaaatagaagtatgtcactctggtaagagatgataggtccgatgactgctaatacttttccaaatggccttatttggatccttcttagaacttttatatttttctaatattgacctacccctttggaactagagtcccattgtcaagaactgtgaagaatcttgacattttaccctacttgcaagctagcagttactcagttgtagttttatggatggtggttaaagatatgagactcctgagttggagttgaaggacagtttattagtgcagcaagcagtagcagtgaccagagtattagcttcctttttttttttttgccgcttttccaagccctggttcccatatagtagtgtgaagaggagggctacatgatgcttgtacacactgtggattgcataacagatgcggaatcctcagcttcttacagaatctgaatagtagtgtataataggaagtaagaatgcctttctttgctttggagcaagatactgtctttgtctcccaacactattgctgtaaaagtatcctcaaaaggatagtgcagaccaaaagggtagttgagtgtcttgctcctaagaggtgcagaaacatgagagtctcatagaaaattgtctcccaataatattttctgctcatttctatactattttgtcttaaggcaaatttttttcatgagtataccactctgatttatctgacagaagatagtgaagtatctgttcaaatagttagctggcttttaaaatcaggttatttgctttcttattgttgagtttgagagttctttcttgattctgggtacagtcctttgtcagatgtgtgatttgcaagtattttctctgagtctgtgacctgtcttttcatattcttcaatctcttttacagaacagaagtttctaattttgattactatcaggtttttctcttatgaattgtcttaggaactttttgcctagttgaaaatcacagagtttttttctttgttttgtccagatgttttattattttgtgtcttacatttagatctgtgatctgtcttgcattaccttttgtttgcataagttatgaggtagagttcaggttcattgtttttgcgtatggatatttacttgttctagcactatttgttgaagagactatcttttccttcggtgaactgcctttttacctttgtcaaaaatcaattgcccttatttgtaagtatattttgctggatttattattctgttttgttgatttctgtgtgtgtcctcttgctaatacatcattgccttaaatagtaacagttttatggtagttattgaaattagtgttctcaaattttgttcttttgctgaattgttttggatattatagtacctttgcattttctttataaattaggaatcagcttgttgatagctacaaagatactttgagattttgattggtgttatgtttaatgtacatgtcagtctgaggagactgacattttgccaatattgagccttccaatccatgaatatagttatttttccattttttaggtctttgattattttcatcagtgctttatagttttcagcatgcagatcctgcacatattttgtggaagtgtatcttttccagatgctattgtgagtgctactgctttaaaaatttttgatgtactaacttattgctgatatataaaaatatggtcgatttttacatattgattttatattccacaacttgttaaaatcataatcataaaaccctttggattttctatatagacaacatgcttttgaataaaggctgttttacaaaatttcattttaaatttgtataccttttatttcatttcctttcttaattgcacttgctagagctttccaggacaatgctgaatagaggtggtaaaaacacatctttgctttgttcctggtgttttattactcttttattattagtgttatgtttagagatggggtcttgctcagttgcgaaggctggagtgcaccggtatgatcaaagctcactgcagcttcaaactgttgggcccaagtggtcttcctgccccgccttcctgagtagctgggattacaggcatgtgccatcatgcctggctaagttttttattttttgtggagatgaggtcttgctgtgttcacaggctggtcttgaactccagtctcaagtgatcctcccacttgtactgggattacaggcattagccaccacacttggcctcttattatcattattattattaatatatataaataaatatacatatatttatttattgagacagagtcttgctctgtcagccaggatggagtgcagtgccacaatctctgctcactcaacctctgcttcctgggttcaagtgattctcccacttcagcctcctgagtagctgggattactggcgtttgctaccatgccgggcgtggtggctcacgcctgtaataccagcactttgggaggccaagacgggcggatcatgaggtcgggagatcgagaccatcctggctaacatggtgaaaccccgtctctactgaaaatacaaaaattagctgggagtggtggcgtgcgcctgtagtcccagctacttgagaggctgaggcaggagaatcacttgaacctgggaggtggaggttgcagtgagccaagattatactattgcactccagcctggcaacagtgagactccatcttaaaaaaatgttatgggatgaaattttaaaaagacctttgaaagatacaagataataggattcaattctgtataaggtagagataaactgttgatttgtactagtttgatttgtgaaatattacaattaggctaaatcaaataggtgatgggtaatttgagaattgatttctaatgctttgtcctagatcattcaaaatctgatgttcacataactacttagaactcttgactagttgtctgtgctttttaaaaacctttacctggctggctacaacttttctaccgccataattaaaattgaaaacaaaataattagtctcttaggaaaataatttacgaacactatctaaacatgctagatttaaaactaccagtatttacatggttagaattcatgagcagtcttcattagacttactgctgaatgaccagcatacagtcgctgaattcattgtgcatcttttaagggaagattgttttgcttgtatctttgcagtcttctctgagatctttaatgttactagaagttataaagtttggttaattttcctaataagcctttatctgattctgtgggctatttaggtttgggatgggatctgttgtcttaatttggtcaccattggctcttggcttcaaagtggaccctaaactatattcctagtctgtctagtatttgtcttttttttgctgagatatgtgacccctggggaggtttcccttattttcaataagttaatctttctcttttaggaagaaaagacaaatttctcataagggagggattttttccttttttgttctagagtgcctttcaaattaacaattttgttcatatcaaaagttgcccataatgatcactgtaagtctcaagttattcttggtgaaaatatgccatttagaaagataagtatctgaattggaagaagcatgtttcatgcttggagaggttgtggagttagactgacttaaaaagtcagttttgtgcagcctgggcaacataacaagacccagtttctatggaaaataaaaaaaaaattaggcaggcgtggtggtgcacacctgtagtcctagctactccagaagctgaggtggattgcttgagcccaggagtttgaggctgtggtgagctatggtaatgccactgcacttcagcctgggcaaaagagtaagacctcatcttttaaaatatatatacaggtttttcttcaaaagattccaaaggtactgctttaaaaaatgtaagattttctaagcaacagggccgagtactttgctttaaagtttttatgaatgcctggcttggctatctggttgcttttgaaatcaacatcttactaaactattaatgcttttaaaatgtgtgcagaattacatatttgtaaatttaacttgagtctgtctaggaaagcattagcaagacttttgtttttgtttttgtttttggagacagtcttgctctgtcgcccagcctggagtgcagtgcaggtcactgctcactgtagccttcacctcctgggctcatgctatcttcccacctcagcctcctgagtagctgggactacaggtgtacatcaccacacccagctaagtaaaaagatgtatttttcatagagacggggtctccctatgttgccaggctgggcattagcaagattttacgggaaattttttttatcattagtagaaaataataaggaatcccttgctggtaaaatttatattgaaactactcttaaacatatttatataaaatgaccagagatatttaatttacctttatataataaatagaaataaattgaaatacattattaggagattcagattttttaattagtaaattagtgtgatggcttaaagttattgagaggtaatttttcatctttgattagaaaaacttaaaaattgtataatttacatacacaaagtatatatgagctttttatattgatgaactttacaaaatgaacacacttttgtaaccacaacccagatcaagatatcagcttctcaggagcttccctgtatctgtcatattcctttacatgaaaggtaattaatattctgactttgtaattagagattagcttggcttttttttgaatttttataaatcataaagtatataagactatatgatttataagttttttcaaactggcttctttcccacagcagtatgtttttgagatggatatttggcttacagcatttttcattttcactgaggcttagggtttcattgtgtgaatatccttagtttatttctcccttctgctgatggacattcaaattatatcaattttgggttcttacaaatagtgctgctgtgataattctcgtacatatttttttgtgcatatatgtacacatttccattgagtgtatgctcaggggtagtatcacttagtctttgggtttatcttcagcttagtagacacttccgaacagtttcccatactgtttgtattatattattatacatttttacctgcagtattttagaatgtcagttgctacagatttttgcttacacttggtattgtctttttttagataaaagttagtcattttggagggtagtagtatgtctttgtgaagttttgtttggtctttagcctatcttaaaaatcggtttgttttttttgttgagttgaagtatttttaaagaatatattttgggtatgagtctttagtggaacatgtgcattgctgatattttctcctacactgtagcttgcattttcatttttaatttatttaaattttattttattttttaagagacagggtctcactctgtcacccaggctggagtgcagtggccttatcatagcttattgcggccttgaactcttgggctcaagcagtcctcctgcttcagccttctgagtagctgggactgcaggtatgtgccaccacacctgggtaatttttaaatttttttgtagagacagaatctcactatgttgcccacactaatctcggactcctggcctcaagcagtcctcctgcctgggtctcccaaaatgctgggattacaggtgtgagccactgcgccagtcatttccttctttccttctttctctctttccctctttccctctctctttctctcttcctttctctctccttccttccttccatccttccctccctccctccctccccattcccttccccttccctccccctttccctccctgcttccctccttccttccctccttccttctctctttccttccctccttccttccctttttccttccttccttccctccttccctccttccttctctccttccttccctccttccttccctccctgtaattgtaatgaaattgtttgtttgtaatgaaattcagtttttttatgtgctgtgtattaaatctatgcctaaatatcgtgacagtatttatcttgtcactatataagctttattatttaaaattttatatatataggtctctaatatatcttattttttttcccaccttttctgtggcttgtggatagatgttattcattttactgattttgattttaacagtagtagtcatagaaaatctattgatgtggcttactcatgagaaagcatttttatttttatatgtgatattataatttctagtatggcaacattttctgctagttatgatatgtgatttttactctgcagattctttaagaggaatttaaaaacagctttattcctgactttagagaaggcagtcagttttacttaatatgtcattttatgtcttatttgttatgttttgtttttgaggagtcatactggtagtttaaaaatactgagttttatcatcaaatgcagctacaatgtttaagcagatgacttaatctccgtgaggcatgaggtgattaaaaaatgtatgtatatgctttttcaaatacagagtaaattgcctggcagacaagaagagcttcataaatattatttagtgctttttattctagatttttgaaataaattggactcgacttgatgcaaaggatttgtactataagtttattataaaattattaaccgctagcttttgtaaatagtaaaattgatttgcccattatacatttctttttgttatgcataaaatattttaatttttaagtaccaacataggatggatttttaaatgcttcctcatgttaattttttaataaacatagaatgaatactgtgtgaaatattttcccactttattggctctgttttaactcagtagactctatagttagattgtctaggtgccacttaaaagatggtaactagataccagaatgtgttacattatatgttgattgtcaggaagaactgaatgcatgaatgcttccctaagacattgttagcatgccgtggtcttgatctataattttttgtctaagttgtgatagagctcattctttacatggtctagtaaattcagccaatgtctttataattcattagcatctctatatattacctataaaatttaaattataaggctatgaaaaaattgtttcatatgtataatataccaaagttttagcatatggtttggattttaaactgttttactgaaacaaattaccgtcattaaatggaattcttaggtagacattacagagtaggtgtaactctgaagttgaaaatggtttcatcttcttttttaaaaaattttattatatagggaatctcaaccaccagcaggattttaaaaaggctatctaaatatttggtaagtaaatattctccatgttaaatattttgcgtgttacttaagtttacacatatgctacatgaatgacatttacaatagtgagtgtaaattatagttataattaatattttaaattttacttggttactagaatttttgtctccttaaacctattccaatccttttctctcttgttctttatgttgtgtccagagattctttcagtgtacagccttattattaagagttcaaggaaagaaatggttttagtgagcaggaatgctaatactttatgaataaaacaggatttcccctacttgagattttgtagtatttcttttttgtgaaaacactaatacagatttgttctttagccatccattgcttgactcctccttgtatttaggtcctgtttgctgcaacatgccaacatgaaccaaatactgtggtcagggtctatgcatttcctgtttagattattctttgttccaagcttaaaatatgaaaaattttgtaggtgtctgtagttaagaatttcataaacttatgatttcatagataaagcttttacttttttatttttgagtaaaggtaggtgagtcaatctcagaatgtattttacttcaactacatagtattttatacctgtgtactatggtgattatatagatataaaatgatttggttaatcataatagattttaaagttattaaatatgcttcagaatgggaaagaagtgctgagacattgcataatgaggtgtcatagtataggcttttggttgtttttaatatagtcaatagcagattattaaggaggaaatatttagtgataagcattggcttcttttattatactttttaatgtgtttgaaacagcaaatatttgaccaaattatttttcttaaattttatagtaactacagtaggtgcctaaatgttcaacagttatactgttctgtttactgtaaatttgtaataaatataaatacttttaggagcaaatgatgccacagagatctcttaaacagatttttactactttagaaggtggtaactgatttctggagttgtattaagtacaaaagagtaacttattgtcatttttttccctattgatgcgtatatttgagttagagggaagcagtcgtctttgtgttatatgcttatcatgtatatttcatcttagcaaatttattaattttagtgacagttttattgagatgaaatttatataccaggagatttcatctctaagtgtacaattcagtgatattttaatatattcaccaagttatgcaactaccagtactttgtaatcttaggttactttcatcatccttcttctggacgccctctatcacccagccctaggcaaccactaatacactttctgtttgtataggtttgcctattctgggcattttataaaaacagaatcataaaatatttgtccttttgtgtctggcttctttaatttagcatgatatttaaagcttcactcatgttgtagcatgtatcagtgtttcattcatttttgtggctgaatatttctttgtatatcatttgtgtattcatcagttaatgagttgtatccacttctttttttggctattaggagcgcttttctgtgaacattcttatataagttttgtgtagatacgtttttgagtatatatggatggggtgggattgctcgataatatagtacctgtgtgtaactctttgaggaactctcaaaatggctgtaccattttacaataccaccaacaatgtatgaggattgtaatttctccacgacctcataaacacttattgtcagtcttttgtatttcagccattctagtaggtatgaagttgtatcccattgtgattttgatttggataatgactaatgataagcatcatttcacatgcttattgaccatatatcttctttggagaaatatctgttcaactcctttgcccattaaaaaaaaaaagattatctttttaatgttgaatattgtaaacattctttatatattctggaaactagtcccttatcacatacatgatttgcaaatattttctcctatggattatctctttacttttatgatggtgtcctttgaagcagaaaagttttaattttgaagttcagctgatctgttttttgttgcttgttcttttggtgttatattgcagatttgtttttaaataaatactcactgatagcctgggtctatgacaaagttttaatcgtcataggactacgaaaaagcattggcatttcttgtgtttgacagtcaaagcccaaaggaggcaattatccttgtatttgtgcttcagttcctcagctaattgttttaagcaaaaccttacgttttgatcccatgtgttactgtgaaaatattagctgtgtgtgatatgtttattgatattagtcttgtgaatttatgtttagttttttttggattgaagaagggaggggccatccttaatagatgttattagtccgttctcacgctgctgataaagacatatacccaagactgggtagtttataaaggaaagaggcttaattgactcacagttcctcagggctggagaggcctcaggaatcttacagttgtggcagaagaggaaccaaacacatggtgacagcaaggagaagtgcagagtgaatcgggggaaaagccccttataaaaccatcagatcttgtgggaactcagtcactattatgagaacagcatggaggtcatcatccccatgattcgattaccttgcactgggtcccaccacaacacttggggattgtgagaactgcaattcaagatgagatttgggtttggacacagccaaaccatatcaatagtttattatgacaattactgcatattttatttcatagtttaagaaaccattgctttttagactaaggattatcaggttcttatctttcttgtgaagaaggaatagattttgataatctcactgattttaatcttgtacagattattattattattattttgagacggaatctcgctctttcgctcaggccagagtgcagtggcgcgatctcagctcactgccagctctgcctcctgggttcacgccattctcctgcctcagcctcccgagtagctgggactacaggtgcccgccaccgcgcctggctaattttttgtatttttagtagagatggcatgtcaccatgttagccaggatggtctcgatctcctgacctcgtgatccgcccacctcggcctcccaaagtgctgggattacaggtgtgagccaccacgcccaacccagattatttttaagcaatgatattttggtgtttttgtaaacttatgtatggaatatgtaagtttttcctctattaagtaaatgtctttaatttttttttttttttgaaatggagtctcgctctgttgcccaggctggagggcagtggcacaatcttggctcactgcaacctctgcctcccgggttcaagtgattctcatgcctgagcctcccgagtagctgcgattacaggcatgtgccaccaaacctgactaatttttgtatttttagaagagacggggtttcaccatgttggtcaggctggtctcaaactcctgacctcaggtgaccacctgcctctgcctcccaaagtgctgggattacaggcttgagccactgcgcccagccagtgtctttaatttttaaggtaccaatttagttccttattttttatcgttatgtgacgttatgtgatcagttgaaggtgtatttcatgtattttgacctataatgttgtctagtttagtttctggagaaatggtgtgtaacagtggaatgtcacttgtcttcaaagcattagctttctgtgtaaggttgaggttgtaatataaatgcgctagatgtgtttttattaggggaattgactattcttacctttcatgttatttgacagtattctttgtcaacttcaaataacggcctattttgatgagattttatagtgctaggatcactgatattcttgttagttgatttaaaatcatggtgttcattggctaacagtcacttgagtggctattagatgggtaatattgttctcttttttttttttttttttgagaaagagtctcactctgtcgcccaggctggagtgcagtggcatgatcttggctcactgcaacctctgcctcctgggttcaagcgattctcctgtgtcagcctcctgagtagctgggattataggcgcatgccatcatgcccggctaatttttgtatttttagtagagatggggtctcaccatgttggacaggctggtctctaactcctgacctcaggtatccacccactttggcctcccaaagtgctgggattgcaggcatgagccaccgcgcctggccagatgggtaatattgttctatacattgatattcttatggtttatgttatagtattcatggaaatttagcaatggaaaaggaaatgaaaaacttattaatgatgttgttaaattttcaattgtgatgacagtaaggaaaagacataattgagagctacctccaattgtttatatcaaatgtggtaattaagaggattttggtgacctatttatggctgaattaaggcaaaatagcttttatatccgattctttcctcttcccttctcttgttctgtgtgcttactatcataataattgagtatacattaattttctttaagtatttatattttaaataaggttttgatgtcagtagagacttttttttttccttgaaggtaagtaccctttaaaccactaatttgtcactagagtctatagtcgcttccatatataataggtagcacagcttctcaggtcatgtcctgctttgctgctctgctgaccaataatacaccttggagatactggttctggttatatgaatagaacaattaaattgttcttcattagatggatctttgattactaatcttactcagaaaggctcaactggacttggattattctaattgccaatactgtttttgcacaaatgtctgcaaatcattgaacagtaatactgacccctttttcttccaataaagttattgcagtaatcacatcattgcagagaatatttcttaaaagcttttttcaatatttacttctttaatgaaaaacttaatccagattaagccacatacatagacgtcttgactttattattttgaatacctgagatttccaaaatctctttaactgtcttcacacaatttctagtctgtcattttaattaattacaactgttcatttcttctgcttttgtttcctcttcatgtgctgcctagcgttgctagagtttcatcagtttcctgccttgagaggtttctagtacaaattaacattttcccttcctagtttatgcaggttccttcctggtaatttttatctttttgatctgtttcattctgcatgttagttatttggaaccattctactgtgctcaaatgaacagtcctatccctagttctcttattcctttttcatttcatattttataccctttttcctcagtctgtcttaaagaataaagtgttttcatttcaaaagcttattatctctgtttttaatcttagcccttctttcctctactatttttcttcctcttaatgctccatgctgggttctctgccttatcagacttaatcttgaaaagtacgttacttccttcccattatctccaaggttgttatagtccattctaggtgtctccaatttctcaactcttactcaattactttctgaagtttgactattatttctactagtgttcagctttcttaagtgtaagtaaacacatttcttacttaactaggtagataaacattagctggacggatctggccgtaaacatgctattatttccaagataaaactgagttccaaatggctaaatctttgtcttttcacttttcatccattcctgtcttttttagcatttgtttttttgctgcttaacattcacttctcctttgtcttctgtaataaaccttaatggtttttctcctctctctggctaaatgtttgttttctttgttactgctttcttcttttatataccacttatatataaattgggttgaagctttgctcttagctctttttcattacacatcattttgaggagatggtctcgtgttcattatgtagattatcacaaatttgatgactcagaaataccacatttttcttagtgacctgttttaccactttctcagtcgccaggtccttagcaccccaaaattgttatttcccagtggaaagtttgtcttgtacaatgcttgctatatggttggaactaagtaaatgctttttgaatcatgaactaactccttatctgtctttttttttcttaagataatggttttaactgtccacctattctcatgtcacaagccctgtaatatctctgaccacttcttgtctacacttgttaatattagttgtcatattttggtcctaagtttgactaatgaggaagatgacatttttgtctgcagatggtggaaataaaaatcacagagattgtgatttccttatggttttgtgggtaatggtggagtttaaacttacaacgaagtttctggtgacatgtttcctagttttcacagaaaacattctttttttttttgagacagaaagtctcactgtgtcgcccaggctggagtgcagtggtgtgatgtgtcggctcactgcaacctctgcctcctggattcaagtgattctcatgcgtcagcctccaagtagctgggattacaggcgcccaccaccacgcccagctaatttttgtatttttagtatagatggagtttcaccatgttgaccaggctggtcttgaactcctggcctcaagtgacccacctgtctcagcctcccaaagtgctgggattacaggcataagccaccacacccagccaaaaacattctttataatgatacaagtaatataccagacaagaaattactcagtgtactatgtgagattaaaaaaaaaaaaaaaaaaagactggaagtggaagtgggagtacttcaaattcttgtctgatgaggtaaagattttaacttggtggaaggaatagaaatcaaggatgtgagaaatttttcattaattagaatttcgagattcttcttttaagaatgcagtgatgctagtgaagtggttgagtgaaccatctttcagctaacaattataagatctggacaaaatattgaaagaaaaactttaactgttttaaaagccatggaaagtaaccaaaaaagcaaagccagatgagagcctccaactgcaatgtgtaattgtatgtttgtggctttcttgccttatggtgcattttcgcctcctgtctttcagtggcataggaaagaagttacgggtagcctggcagttggaaatttactcaggggaatcatggaagcaataagtaagatccaaaatctgagtgtaaactctgtccaaatcatggctaatcacgaaactatacatgcataggggagaccccaggggacccagtgtaaaaacaggcagaaacaagagcggaatctgctcctgaaagaattgaaccctgtgagatttgtgattgcttctttttttgacagtacatttctcaacttgcatgcaatttgcgtggccaacagctggcttgaggtatcagagcacagaacatattgttgacagaagagttaaaatttagggaacaaacactgaaagcaagataacatcagaggatgtaggccacacatctcagtataatctctgcccatttccttcactgaccaccagactacccaggtgcagaggggatgccctgggcatcaggttagaagaaggaagcagctggaaggtgaaagaactaagcaaaatcattgttgcttactataagggagacacacagtaagtcctcacttaacattattgataggttcttggaatctgactttaactgaaacaacgtataacagaacatttttttctcatcagttgtataacaaagcagtgttaaaggaaacgacagtattcaaggaccttgctgtttgtgttttgcttcaagttgctgtttccaagacctatcgatggtattaagtgaggacttactgaagtttgcagtttgagtccatacgagcccattagaatcatacaacatgaaaaccaaatggtcctttgaaagattgcgacaaaatctggttgctataacttgctatttacaatgtgtattttcaactaaaaattattagatatgcaaataaagtggaaatatgactcattttcaggtaaagaaaatcattcaatagaaattaaccccaagtatagccagatattggatttagcaagcaaggactttaaaatagccctaaatataatcagaagaatttaaggagtcctatgttcaaaggattaaagaaaaatacagtcacccctctgtttccatgtttctgcatttgcagattcaaccaaccgtggatcaaaaatagttgggaaaaaacataataaaatttacagtacagcaataaaaaataatgccaataaaaaacaataaagtcttgttcagtgaatagataggagatcaaaacagagaaacagatactgtaaagaagaagcaaaagagaattttagggttgagatcagtaactggaatgaaatttttatattatattttattttattttattttgtggtggagtcttgctccgtcgcccaggctggagtgcagtggtgcgatctcggctcaccacaacctccgcctcctgagtagctgggattacagacatgcaccaacatgtctggctaatttttgtatttttagtagagacagggtctcaccatgttggccaggctggtcttgaactccctcccgacctcaggtgatctgcctaccttggcctcccaaagtactttgattacaggcgtgagccactgtgctcggccaagcaaaacagttgtttggagatggcaaaagaatcagttaaagatagattaataaaagtcatctatttgaaagagaaagaatggagaaaaataagcagagtttgagagacctttggggtaatacaatgtttgaacatgcatctaaatggagtctcagatggggaataaataatggctgaaaacccccacaactttggtggaaagtatcaatttacatatccaggaagctcagcaaacttcaagcaggataaacacacacaaaaaaacagatgttagcacataagtggtcaaattgctcaataccagagaatttcttgaaagtagccagaaatatcttaccagaaacaatggcgacctctagccatggatatggtatattcagctgaaaggcaaaaagctatcaaataagaattctgtgttcagctagaagtgaaggtaaaataaatacatgttcagataaaccaaaactgggaaattttcaccagccagccaccattgcaagcatttctaaaggaatcaatttcaagggaaatggcaccagatggcaagtaccatctacaggaggaaatcaacatcaaaactagtaaatacataatttactctaatttttataaactatatttttccttattttaaaaacaagtacctgtgacttgaagcaaaaattatgatgctgtattgttgggtttataatggagtttgggaatttacatattgtacaatttttaatatgtaatgacatacaaattaacgtgttaatagtcttctaacttatgaacatggtatatctcattaaggttattgtttaattttagtaatgtataataggtttctaaaaaacttaaaaatgtggtaaaatatgtacaaaataaaatttgccattttagctgtacaatttggtggcacagttgcattcacagtgttgttcgttcattactactttttccagaacttttctatcattccaaacagaaactctgtacctactaagcagtaatttcccatttcccttccccgagtctctggcagtgtctaatctactttctgtctttatgaatttggctattctgtatttcatatatagtagtcccccttatccacagttttgctttccacaattttggttatctgtggtcatccatggtctgaaaataggtgattatagcacaataagatgttttgagagaccacattcatataactttattacagtataattgttcttttttattattgttgttgttaatcttttactttgcccaatttacagattaaactaataagtatatatgtataggaaaagacatagtatatatagagtttggttctatctgtggtttcaagcatccactggggggtctggaacatatgctctgtggataagtgggggactagtgtacttcctgccctaccccttggtttggagtcgctgctgtatgaatataagggcagtctgcctgtgatgtgactctccattgatcacctgggtgtatgaattaattgctgtctataaagagtcttggaatgactattgagtttgctctgtgtatgtatacatacaacagtatggctactgttgtagctgatttggctatgatactgtagtatcttatttgctccaaagagatggagtagtgatgaaatctggtttactaggtggaagctagtgtaaaaatgggtactctgttttattgaattagcttgattggaaaaagtgaagtgctgatggttttgaaaatatgatgataatgatgtcatccttctggtttaaatattttgtagcacttgtggtagattgaatgctggtgtcggtagtaaagtcatgctgcagttatagtctgaaccagctgtactgttttgggtagtaacttagacagtagagaacaccacttttctaggcagggctcctcacctctcctagggggccatttcactgcatcttggagtgaatatacagagaggaagtagctagatcctaatttctacaagttatatcagttggggaacagttgtggttgtcaacctgtgttagggctgtattggttttgctttcagttgtgctataaagtggaaaaaattgaattgtttatttatctcttattgtgaaactttcctgtggcccatagaagtggcatagcaagctgaacatagctgggtttgttcttcattgcaagatcctacccccacctccctttctttcctgcctggtttcttgtgtccatactgcaagctctttttcccagttagaagtaagttagttcactcttaatagagctgatttacaaaggaattttatgtgtgtcatactgtttgattctctgaaaggtagatatgggactgtggtaacaatccagcatgatgttaactgtgctctcatttttaaatgtgcaaatggatgtatgtgaaatggtggtttgtctgatacaatattggctgctaagacatgtctgacctagagcctagatgtgttggcttcttaataatgctggatgatgtatatctggatcattctttttaattgactgagatgatgcgtatcttctacctcttgagagttaggaatgtaaagggcaagtgaaaaatttgttagatgctcttaaaagatgaaaatagatgtgctccatcactagtatagtttctttttgaccactatgtcaacctgtttagaaagtatattttaggccgggcgcggtggctcacgcctgtaatcccagcactttggggaggctgaggcgggcggatcacgaggtcgggagttcaagaccagcctggccaacatggtgaaaccccatctctactaaaaatacaaaaattagctgcgcgtggtggtgcgtgcctgtaatcccagctacttgggaggctgaggcaggagaatctcttgaacccgggaggcagaggttgcagtgagctgagactgcaccagtgcactggcatggcaacagagactgccaacagagcgagactccatctcaaaaacaaaacaaaacaaaacaaaaaacaaagaaagtatattgtaaacatcaaattaaaagaatttcctgaagtaactttttttttttttagtaggggtggggaagatatgagtagaagagaaatgaattggaaactgagtaccactaccctttttcttaccttctatccagaaatctttcttaaattccacagtatcagtgtaacatcttttatcttttgagctgtctttgagattctttactttgtctccagactgtttgttaggattctactagagaagttgttttcagattttaatttctctgctccattttaatcttctaattttttaatgaaaaaaaatccagttttattgagttcttttttttttttttttttttttgagacagagtcttgctctgtcacccaggctggagtgcagtggcacgatctcagctcactgcaagctccgcctcctgggttcacgccattctcctgcctcagcctcccaagtagctgggactacaggcgcctgccaccacgcccagctaattttttttgtatttttagcagagatggggtttcaccgtgttagccaggatggtctcgctctcctgacctcgtgatccgcctgcctcggcctcccagagtgctgggattacaggcgtgagccactgcacccggcctattgagttctaattaatgcataatttgttgagttttgacgtatatgtgcactcatgaaaccatcaccacaatgtatatatccagtgaatatatacatcacccttaaaagcctctttgtaatctcttcactccccacttcgcaggcaaccactgatttgctttctgttactgtaggtcagtttgtatattcttgaatgttatgtaggtagaatcatataatgtgtctcctcttttgtctgacttctttcaaccctagctcaatatatttgagatttgtctatattgttggatgaatgatcaaaactttgtttttgtttttttaactggggaatagtatttcatttttagtatatagtacaatttattttttgcccatttccatttagctgttattgctggattgggttattaacagttattgactattatgaataaagtggtcacaaatgttggtgcatggttttttatgtggacttgtgctcttatttctgctatgagtggaatggctgattcatatagtaggtgtatgtttacctgtataagacactgccaaacttttccggtttgtatcagtttatattaccacttgcagtgtatgagcattccagttgcttcacatcctcagaattcttggtatggacagtattttaatttgatttgttttagtagctgtataataatgtcttattgtggcattcattaatcattaggaaaatgcgaattatgttgaacatctttacctatgcttgtttgccattcacatctttttctgttgaagtattttctcgaatctttgcttattgatttattgatttatttattttgagtaagagtcttgctctgtctcctaggctggagtgcagtggtgtgatcatagctcactgcagccttgaactcctgagttcaagtgatccccctgcctcagcctcctgagtagctgggactacagatgtgtactacaacacttggctgtttttttttttttttttttttttttttaaggatttttttaaagagatagggcctgactgttgcccaggctggtctcaaacttctggcctcaagccatccttccacttcagcctccagaagtgcagggattacaggcttgagccacagtgcctaaattttttcattgtattgtttgtcttattattgaattataagagttctttctatgtgctaaatactagtcctttggataattacttgcagatttttttcagtttgtggtttgcctttttttctttacccatgtcttctcaagttcaagtcttttattttgatgaatacacatttatagtttttcttttatatttcatgctttttgtgttgtattttggcaggccaaataatgacccctgaaagatgtccatatcctaatttccaaaagctgtatatatgttacctgatatggctccacaaactttgcatatgtgattaagttaaagattttgaaatgaggagattagccaggattgtccaggtgagcccagtgtaatcagagagtccttgtaagaaggaggcaaaaccaatcagggcagaagagatgaatgactgcagcagaggttggaatgatgtgctttgaagatgaagggaaggggccatgagctaaggccatgagataataaatttgtgttgctttacaccaagtttatagtaatttcttaccacagcccatatagattttgcctgtaagtggaatgccgctgtaacaaatacctaaaaaggtgaaagtggctttgaaattggggtattggcagaagctggtagaattttgaggaacataatggagaaaacctagattatcttgaatgtacagatggtagaaatacagatgttaaaggctctgctggtgatgccccagaaggaagtgaggagcacagtagagaaaatgtgtatcgtcttagagaatacctaaatcatcataaagagactgttggtggaaatgtgaacattaaaggtgctgctgcttgtgagtgctttgaaggaaatgaggaagatgttattggaaactgaagtgaaggagatccttgtttagattgtaacagaaagtttacctgaattccgtcctgtagttatgtgactaactctcctgtgttgcctgggtatagcagcaatcatttatacatacatttgcagttctgttctgtacttgttataaagtagttttaattaaagtgacagatttatgtttttataaattaaatttatatttaaaaaatcagtatttagaacaaatatcttagtggactatattcttgagatattattattaaagtctttttacagcttcctttcaaataaatggatatgtaatttaaacctttaatttctggatttcctgatgacttttctttaaaaagaataatttttaaaaacacattttaatttataactaaaatggttatttaaggaaacacatatattagttttatttagatatatgcttttttattattaatttggaaagtggaggtgcattgtttggtagaataattttaaatggtagctcttgttaatggctaatatttattagtggatacaacttacaaatatctgtacattcagtctttatccttatcttccatatctttttcttctgcattctaggtttttttgtttgttttttggaaggaggatatataaagtaattattactacatttttagctgttgccaagttgaaagtcagtgtttagttttttttaaaaagggctatttagtgtggaattcctaaatattatagttccctcttctgtcctttcagagctattgcaccctgttaaattttttttgcattcagttcaaccagtgtttgaaaattaccaatagacttaaagtacttctctgaagttagaagagctcctatgtctgatgctatattgctagtatttctattcaggttggaatttggaatagtcattatcaaaagttatttgtaggcaaaagaaaacaaaaagaaaaaagttatctgtaggaaatattggagactggggtacaaggtaagtgacacagtgaagaagcacagacaatttcagaatatgagacacctaacatggtttctgcaaggtattggcgtggaaaaaaaaaaaaaagggggggggggcttagagagttactctccagtaaaagagatataagaagcagtactatagttatatacaaagggtagttctttggattctgtttagatcaaattaactagaaaatacatttttaaaataagatggggaatttgaatattgactggtattacttaatatcgtggaaatatacttattttgaatgtgtatagtgactttgtgagtatgaaaggcagtggccaaattatttagtgatacataatgatgtatatggatgagggaagtaatgacgtgatgtctggaatttactttaaaataccttggaaaaaatgaataaaagatagataaagcaatattgctaatatttcagtacctgttaaatataggtgacagtatatatatagaggttcattatactcctttctccacgttttgaaaaatttcatttaaaaattcaaaaaaattctaaaaaatattttttcttttagaaactaacacatgctgaaaaaattcaaattttgttcactgaccacgtttttgctgccaccactctttcaacatttaaaaaatgttcttaaatctttaaaaattcgatttacattttcattaagaaaatgaggcatttgctggccatttcatccttcctcttgtattttttctccttacctgctgccaccgtttactagaaaaatatttctcttgttttttctgtaccttctccttgaaatataaaagttcagtgaaggcaggagagattttagcccgtttttgtatggctgcatcttccttatccatacctgcatagcatgtggtaggtgctgagtaaatatttgaatgactgaatgggtgactgaatagactgaatgaaccagagttgtagaagacatggggtgacgtggggtttggctaaggacagaaccaaggagaacccctttgaaaattcactctgtgggatttacaggggaaaatgtgggctactacataagaaattaagataagaaatcatctttcctgtttgactgtaaagccttaatatttcaagcatttaacatattctcagcataaataattaagtttttttcttcttttttctgaaacagtctcactctgttgcccaggctggagtgcaatggtgcgatcttggctcactgcaacctccgcctcccaggttcaagtgattctcctgcctcagcctcccgagtagctgggattacaggcatgtgccaccacgcctggctaattttttgtatttttagttgagacgggggtttcaccatgttggccaggctggtctcaaactcctgacctcaggaacccacctgcctcagcctcccagagtggtgggattacaggcgtgagccactgcgcctggccagtaattaagtttttatactgtaagttctctaattgtctttaatgtattcttgaaagtgttttcctcctaatttatttattactgcaaggcaatccgttcttgaggttctatttaaagtttatgtatttcttctcaggaaaaaaaattacttaaaactagtggtttgtacagtcaagatgagttttagaagctgttcttataatttctttttatgttaaacatatataatgtcacatttcccttttcctaacaactgatcttctttctttttcaacgtgtatttataagctagatttttaaattttgctccagggactgctgtagttgttctactacttaaaaaaagaaagatgttagtattgaacactattctgagacacagctgataacaattgtgctcaacaatgaagatggctaaaaattgggttttaaaaataacagtgaaaattcagaagcattttatacttgctattctaaagtgagtatttttctaatctctgctttaaaattactgaagtccttttaatgaccaacgctgtattttaaggaaaaaatgtgagcaaagatttttagtgattctaaatttgttttgctctctggatctctttaaacttttaaaaattattgaagaccccaaaaagctttgacttatgtgggttatctctcttgatatttaccctgttagaaaataaagctgagaagtttaaatagttttcatttattaaatttatttaaaaataacagctaattacatgtttacacaattaacaaagtctggcttacaggaagacagttggatgctcatatctgcttttgcattcagtttgttaggatattacatgctctatactctgacaaaaactttactttgtgtatactcaagagacagagtaaaaaacataagtaacatcttagtattatagaaataattttgatcttagaaactccatgtaagtgtctcaggaactcccagggttcatattttgaaaattgctggagtcatctctcagaggctatgtgtgacaaatggtgtttttaaatgaaacaataatttttaaaatatagtgtcaattggctaagtttttatttgatactttttttttcttttttttttttgagacagggtcttgctctgtcgtccaagctggagtgcggtcacagctcactgcagcctccacctcctgggctcaagtgatcttcccactttagcttcccaagtaggaagtaggtgggactacaggcaagtgccaccatgcctcagtaatttttgtatgttttgtggagacagggtttaccatgttgcccaggctgctctcatactcctgggctcaagcagtctacttgcacccaactcagcatcccagagttctgggagccggattcttatttgatacatttttacctttaggggaactataaaaattagcttatgcttatttatgcaaataaatttgagcattgaggaaggatgtctcttgttcagggttgtgtttgtagatttcacatcttttagactaccatttaagagaagtgatcaccttgtatcttaaggaaatgaaaatcatttgatagaaatggattgttaaatatttttaaaacaagttttgacagttacttgcaattaaaggggaaagcaactttaaaatgcattagttaattgaagaaatactcaagatccttaattgttgttagtgagcaagtattaatgttctttcctctttgaaaacgtatctgtacctagacaaagttaattataaactttttcataaacaatattatgcttctttttcttctaatttttaaaccttatctttgttggtttgccttccagctccatctatctgcaacctaagaatcaacaatactatacatcaaattagctgatgtggaaggaaaatgataaataatgaaaatacgtcatattgcttatactctaagttataattaatataagatccaagggatattggtgtgggggacgaggaggaaggaacattgcaagtcaagctatttcacaagtattctatacctttgaatcttttatttcatagttttctttagaaacaatagtgatgcagactgaatagctagtaagataactttcattaatagcagtatggcagggatttttaattgatgcttgttggtaatattagacacatgatttatttataggcttttaattagaaaactaatacaaatatcaaattgttatggacaggttatacattttttggcaacacaaatcctaccaggttttaatgcctggtacttgtttttacattagtatgtggtattaattttttcattactactcttagcttccctagcttacccatttgctaggagtacatagcagcactaggacatttttcgctaacgtggctggcatgcatctgaaagtgtgacagagcaggggtatagctagattttagaagttcttttgctcatttaagaaacttaaacttcagatttgatagtacttcagattctacataatgtgctctttcgatgaatagctgtgtagcagcagcacaggaaaagcagagttcttggcaatacccagttcaattgcatctgcagatgaggatttaaaattctgtgcagcagacagtacctccagcaggcgagtaaaaggttactgcattatttttcttgtttgttaccatagcctttatctaccaaaggatttttaaaaaattgaatgtgaagtgcatgcctgtttttagatattctggaaattgatttaagtataacatgaatatcaaaagggcagtgcaaggtgaaggcagaggcagtgctggatctttttagctttaaaccagggaagaaattgagcatgttacatacacaaagaagaaacctttcagtgtcacagacaatgggaagttttaaaatacgtattttaattcaaggtgtttattatttagttttagactatcttccccaaaaagggtgctcttacattagcaatcattggtctatgaatgttcatttaagttacagtaatttgaagtatgattatttgtgaagactataaagtatttgtattaatgcgaccctcccttgtcctggaaattgtaatgtggattaattacattgtataaacaaatacctttgtgcattattggcaaaggtagaatgcttaagtataaaaggtatagtatagctagcatacttaatattgttgcttatgttttcagggtggtttgtggtttttaaaataatcttttaaataaaatgcagacaagtaagtgggagaaaattcagtatcaaaacaatgaggtttttgatggctttttacttgtggtcagtacctacctatatagccatatgtccttttttctcattaaaactcttctaacatttatgatagcaggagcctccttggattatccagcttgtttattacatcattatctgcaccagtatttttgctatagatttttattgttcattacttctcaagtctacataaagtatccagagggaatttttgcttgtatattttattcagttaccctcctaccctcttccatcagtcctcaaagatttgtattagctactgtctacattttgtttatttaaaaaatacttaggcctatatttttgtattgtagattgaataataagattgaaaacaattctgtaaattaatctatagtatagaagtaaaatttgttgattattcttactgtgagtatttggcaggcttcttgaattgtagagtcataaaaggtcagcagttctgattggtaagttaaagaatccatccagtaatttgctccctgttgtttctcaaagcaatgcagcagcagttcttttccagatattaaacggttcttgaacagtgtgtgtggagacggggaggggtggagctcattcctgttggttgttgaaatcgtgtgcatttacagagggaacaggttggataggctgagctgaaggagtaggcaaacagatctaaactgatggaagacagaaagtggttagtataattttggggtgtcttgagtttgctcctttgttaagtacttgggctttaatataaaacaatttaaaatattaaagcaccttaccttctttctaaagagtagctgggagacttctgttttaatatccagtttttcttggcgatgagtttgtggctggcatcttctgtagcaaagctgttgttttattcttttttagtagtgtttctttcagccagagagctgcagaatgaggcagtttgacaattttgagtatatatgtgacatcaccagttctgattttttaagtcaaattctcatctaatgagcaagtcaatgtgtggctgtggctgcagcattatttcttctttaatgaagaggttgagccgttcgacctgctgctccgatttgttctcttgtagccatacatcagaccagttgcagagattatccatcgaatgtcccaggcaaccaaaggtaactacatagatttatttcaaataaaaatatgcaatgaaaatggatgcattatgactaagaccaaatgattaaaaataaaagaccaattaaagatgttcttagcagttttcttgaccttgcagtagatatccaatatcattttgtcatcatcagattgtgtagcaatggaaatgcactgcagtaattgattttgtaataggatcaggtgatttactagctgcactgacaaccacttgcttgcttgctctgagctgtggagcactctaatggatgttgtgatttcagcctggagtttatgtgagactgccggccacttaaagcagcagcacttattttaaagattagattagtttttctttcttgttttcttcgtttcaagttttgtgagtagcctcagtaactttatggttaagttgtatgccttcatgaaattttagagattatatattatttcattcatcaattcatagtctttctgctccatattcctagctaaatatcaacatattctggtattgaccatgagagcatatctctaaaatatgagagttattggtaactatgctgtgttatctaaatgaagtggaatattcctcacattcgtagatttcattagcttcagactctagctgtaattagaatgatggtaaggttcttgatctcttgagttgtactgcagttgttttgcatccttttttggtcttttactttcttagtggtttcatgggtaaggcaccatttaggaaatatgagttgtattacttctaagggatactgatgaggatatataaagctattttaaagtagtgtttaaggatatagcaaattaaaaatctaatatcaagtattataaatttcaaagtgattattttaaaataatttttgttttccttttctatgccttttaaacaaataattggttcaaatatagaagtgtaggaatattgctaactgtaaaatagaactactgtcatagaaactcagatgctgtcaaagactttgattacttaaaagttttgctgatggtgttagattagaaaagaaactctcttccactcccttcctcaccaatacctctacctcatgtaaagtgttttatacagactccaccacataaaaatactgaattctttatcattccctgtttctgttcttgccatgatagagacaccatttctctcaaccacatctaaaaacatttacaaaaattaaataagattaacaatttactgtagtagaaacggggcataaaattgtcatcacatgtggtattcaaatcaccatgttaagagaactttcctttttgatgtactcaaatagtcacttgtagtgtttgaagccttagtgtttctagaaagttgaaaatattatctgtgctagtctgcacatttcctttaattcagatactttaaacattaattatggaaaattgaaaataatttaaacactagtatttgtaatcttttattattcaacaggtaaaaagtttatagactctcttgacttccaagaaaaaaacccttctgtgaacactgatgaacataagcatgttaatatcatttaggattcggtcaaggatgtgtctgaatttcatatatattgaaaatgtttaatgatgggccaccagcaaattaatcatggatatgttttactggagtgccgtctatgacagcttcttttcatgatgggttcagcaaataggaaacgaggaagtaaacaccagagtgttgactactttttataaaagttagaaagataactatgattggtctgtgattagacagtattttatgtaaaataaatgggcagcgtgaagttctagcctcagtggagctgccttttctaaagagccctggatcgagcattaaaagagttggatttaatttggctctgccattaatctatttgataaccttgatcaaattatgtatgaacattttaaagtcccttaaacatgctcttaaaatgtccattaaaaagatttcaatttacccttaccagtgggaagtattagaatacttgaccttgaagctatagaagttagagttaggaagaaggatgaagtttcttaaagaatcaagttgtaggtgatgttaaaacctctcctttcactttttatgtctttttttgggggggtgggtgggtaacatgtttttgctaagaatactgttttatctctttgatatccaatatttcctaagtaggatagtaattctggaaattatcctagtggttaatagaatagacctgggattaaaatctggtgctgccaattttttctagactttctaacaaagataatgtcattagggagtttattcagtacctaggatattttttagtaaacacgttttaagaaggttggccattatgttattggtgctttcttcctgtatggcctattagataagcgctgtgcagtcatctttgttgcctaggcaaaatggtttgtaggttcattgattgaactcttactttggaccaagtgctgtactaagcactttggttttttttttttttttttttttttttttttttaaagacagagtcttgctgtgtcacccaggttggagtacagtggcgcgatcttggctcactgcaacctctgcctcctaggttcaagtgattatcctgcctcagcctcccaagtagctgggattacaggcacctgccaccacacccagctaatttttttgtatgtttaatagagatggggttctgccatgttgcccaggctgatctctaactcctggcctcaagtgatctgccccgcttggcctcccaaggtgttgggattacaggtgtgagccactgtgcctggcctgtactaagcacttctatgttaattatgtcatttatgagaaagactctaatgattatttttaaagatgagagaactgaagctcagagaggttctacaactcctaaaaatcacacaactgggaaatagcagaaccaatgtcaaaactttaggcatcagcctgctgctcaaaggaagtgctcattgaagcgcttcggattttgaaatttctgataagtataatgcaaatattttttaaaaatcccaaatctgaaacatttctggttccaagcatttcagataagagatactcagtttgtatttgtactttcaattaagctgtgagtgtagagatgaagccaaatttcatctgaagatgtaatataaatgattacctaatttttttagtcttgaataagaaatgatttgttcacctcttactcagcaataattcgtaggaaaaattattcatataaagcatatttgtactatttggagtaatgttttccaaagtgtggttcagggctgggcacggtggctcacattggtaatcctagcgctttgggaggtagaggcagatgggtcgcttgagtcgagaagtttgagaccagcctgggacacgtggcaaaacctcatctctacaaaaaatacaagaaaattagccaggtgtggtggcatgtgcctgtagtcacagccatgtaggaggatcatctgagtctggcaggtcgagactgcagtgagctgagctattattgtgccactgcagtccagcctggacagcagagtgagaccctgtctcaaacaaagaaagtatggttcaggaatcacttgtatctatcactttggatggtggttaaaagtaccagtttacatcagggcacattgaaagaatcaccggaatgggatccagagatctttgtttttaaataagcctctcacatgattcttggttataccaaattgttacaaccaatgatattgagaatgttttcctgttttaccttgtttctatgccttgcagcttttcctttaagaatttgtttacaaaccatagatggtttgtaaaattatccttctgacttatggtgaaatgtaaattggttcttttgtggtactcattttaggaacttgtttaggattaaaagtattcataaactttgactcagaaaacctacttctaggaattatagagataattcctaaggagatactcagattcgcaggaagacttaggcacaaggatgttcgtaccattatcatctataatggtgaaaaactggaaacaactcaatttcaaacatcagataaatggtttgttttttatatccatttgtttggactaaccatccagccataaaatgttatatggggaagattttgtaagacataggaaagtgctcatgatttaatgtaaagtctcgaagaatataaaattatggtcatacatatatgtacatatagtgcatatggtcttaggttaaatcatatgaaattaccgtttttgtaggtcaagagtagtagaatatcagcattttcatgtagtgtaacctaacatggcacccatttttaaagcacatgtttgtagagaagcacatgtttgtagagaagcacatgtttgtagagaacgctttgtagagaaggagctggaaggaaatacagcaaatttataaagtgattatctctggatgatgatattatggataatttgaaatatttcatctttacatgtcttatgttttcaaattttctactataccttagactcaacctttgaaataggacaaagtaaattaataaaacagggaacagttgcaaactttctctgaaaaacattaaaattttttagaagattgtaaatcctttaagctagtataaggacccctttatactaatattcttaactcttgtattaattattgagtgtgtttatgcaaatggatcatatatgcctttacctacccacccagcaaattttgattggattttaatctgcagtagaaagtgtctttcaaaagaagagaaaaaaatcaattttcaaagtttttaaaaagaattgggttcttaaaagaccgccaactatatgcaggagtcagttgggtagccacgttaagcacaaagccctgttttaggctgtgtggttttgatttttaattgtaatttaactgatcgataaaactctgtagattaaaattagtaatttgtgtatttattttaaaatattactgtatttttttgaaaggaaaatgtttctcccactttcatacactttaatcgtttaattttaaagaaatagcttaattaaagtaacagctaccatattctggttatctgccatacaccaggttttgggtgctttaatatgttttttgttttgttttgtttttttgagaaggagtttcactcttgttgcccaggctggagtgcaatggtgcgatttcggctcaccacaacctccgcctcccgggttcaagtgatactccggcctctgcctcccgagtagctgggattacaggcatgcaccaccacgcccggctaattttgtatttttagtagagacagggcttctccgtgttggtcaagctggtcttgaactcccaacctcaggttatccgcctgcctcggcctcccaaagtggtgggattacaggcatgagccaccgcgcctggccttgggtgctttaatatgttacttctttcaatcttcacctagaatgtattaattagatatgagctttgttttagcgttgaggaggcactgaaactattataagctttcctgagatcatattaagtggtggatctaggtttttacctcagtaatgtctaacttaaagacccatgttcttatccctgatactgtccttgttggtctgtctgaaacttttaagtgttcataacttgggaaacaaaactgttgtataagccttcctaattcagactgtcaaagtgtagagcaaagtatataatgagtcattattgctgatttttattcaactatttgttacctgtcctttaatctggtcagtacatgtgtactggcatttaacgatcgcctgctaatagctaacctcttgtgtaaaccactggaaatactaaaacagagaagccaaaaattacttccttggagtttacagtcctaatgagagagacagacaacaaaatagttacaaggtatttcagaacataggtatggaatagaacctgttggaacagaaagtttttaaactaataatgtttgggagtagtggtgaagagttacttgggaagccatcttggaagaggtgaatttagaaggagccatagatttcgtttttgctaccagcctaggaatttacattttaatacaagaacccctgcctccagagtgatctgtaattctactgaagtttgagaaccaccactgtagattgtagttgatgctacgagaaagcatataataccctgaggaagctgtgtggagtgggaaatgagaagttggaaacctcagagcaacaacattgctttgataagtaggggaagttatatgatagttacgattaatatattataagcaatatcttttagtgcctagaagtaagattggaaatgtcttgaattttgtataagatcacaaaacttacaggaagaatatcaaaattccgattgaggttacttttttctgggagggatggtgaaatgttattctttaccctacaatgtgtgattaagagtgaataaaaatcgtgttaaccttttaaagataatgtttaagaaacaggtttaatttttaaaagaaaagtgagcataggagcaaagttttgtaacatattctgcttctatataggaaattaattcctaaattttggaaatgactagttgaaagtaatagcagtctatcctccaaagagagctttttaaaatttattttttagaatcagacctgggttaacttttagatataatttggcataaccagcaagtcattggttattcaaaaataaagattggaaataattgccatatagtcttggctctttgcgtattttgtgatactgattgttgcttcctcctttacttccattttattattagagcttcattaagagtgaattgaaaagaaaactgaattttattattttaaaaatctgaatagttggattggggcaactttcttcctatttatgagacttcactcatttatgttggtcttatattgacattaaagaatcagtgtcatatactggtgaatattaacaaagagacaagattaagattaaagaaattgaacctttaagcaggaggcgtgtgactaatggagcaaatttctgaaaggcttaggggtagagaaaatcaaagctactgatggtattaatagtcttagaaatgatggagattacatttttcctctcagagacaggcgacaaagaagggaggagtaaagaaacaaaacctttgagattgagatatcacaagttgataggtacacagctctctgaaagcttcagtcatctcaataaggagaggaacatacttagccatataagttcgagttgctgaatatacattctatgtaggtaggtctgtgtaattttgatacgtattttctgtttatcacagtggaaattgttcttgatcaatgtttttatttcaataagaaagatatattgccgcttccatcttaaaatttctacatagaagagacatgacgcttagtgaacgttattgaaaaaaaaaaaccgtataaacttaagcaatgaagaaagagaaacagtgtttcagaatgttacagtattgaacctgaattggtagagagaatagaaagtggtgtgaacagtcagggtccaaatgacattctatataaagcatataggacatgatttggagcagggagtgggatggggaatgcttagattacatctctttactagatgggtgtacttgttctgtgcaaggtaccattttctccccttttttgttagctcatatatcccttcccagttttgaagagtgctccactggtatttataactttagtgatttgacatttcaggatatacctgtttcagaaaatcataagaagttttaaaaatgccttgatgtaaaacaaaatttcaggtaaacttaaatattttaagtttttaataatttgtgttaccaaaattaaattttggttagagtttgacattcctaagtgatagaatcatcttaaacacatgttgtcaacagaaatttgaatgctgaagtcaatttttgttattgttattgttctgcttagtgaagaaatgtatcctctctaaccagggacagtatgtactgctttctccttaatactttgagattttcataaagaaaataatttcaaaggtgttgtgctgcaagctaaagagattatttctaaaggaagaatttgtcattctaatggttgtcatcttccttgtggcattattataaaattaagaaactgaaaaaaaatttttttagaagacatagtatataccagaatttaaatttagtttggcataagaggccacatattctacctatgctattacagtctgtatttgttattgcctaattttgactcattttgaatatctcactccagtcctttttattagtatttcttaaaacaaaaatgggcaatatgttggattgactgaaaataatttttaagtgtttagtagcaataaaatttaatcttttagtgcagattggtttaccccataacagcacatatggaagaagtaaagccaggtctgtatgaagcaggaggtgacattggactttttttttttttttttttttgtgacggagtcttgctctgtcacccaggctggagtgcagtggcacgatcttggctcactgcaagctccacctcctgggttcacaccattctcctgcctcagcctcctgagtagctgggactacaggtgcctgccaccacacctggctaatttttttgtattttttagtagagacggggtttcactgggttagccaggatgtctcaatctcctgacctcgtgatcggcccgcctcagcctcccgaagtgctgggattacaggcctgagccaccgtggacttctttaaataaccatagtacaggcagttacttttgttatataacagtatagttgtctctgaagaaaacctgaagctctgcaaaatcgggccctgaaaatcggtttctgagtggcttgttcctgtgtaaacttgtaatctctgtagtaacgaaaccagtacccattctaataaaaatattatatagctaaatatttaccccagttagttctaagttctaggatttatgctttctcctttgaaatgtaggtcctcgagaacattcatttctacttatgatgaaattgtgaaaactagtaaatctgatccagggtgtagtttttatcagttgcctctcaccccttaaaaaaaaaaattaacgtgggaaaaatattgtcatggattttctatctgtactcacagcttgaccagatggttttaacattgtggaatgcctagcagtttaaagccattaactagcctctggttaccctcttctggatttctagtttttttcttaaggtcatcatgtattgcttaagctctgtctttgtgagaaagcttgtccctgctggctttaaaactttactatgctggggaaaattttggactaaagtgacattcacattatactgacctcatcgcccaaatgatgaatgaatgaactaatgtacactacaagaacatgtcttaataggaaagtagactgttgtctgtagttgtcccattgttttatcattgctgctactatattgacatgaagtagcagtgggtgtgcatgtttgtatattttttctgtgctgttaaataagtccacgcacatctcccatgtgggtagggtagtactgggtgatggagtaggtttaccagtaccatttgtcccttactttacttgtatagctttatgttttaaaatagagtgtttttgtttttttgagacagagtctcagtctgtcacccaggctcgagtgcagtgatgtaatctcggctcactgcaacttttgcctctggggttcaagtgattctcgttcctcagcctcctgagtagctgagattacaggtgtgtgccactcctggctaatttttatgtttttagtagagacagtgtttcaccatgttggccaagttggtctcgaactcctgacctcaagtgatccacctggcttggcctcccaaagtgctgagattacaggcatgagccaccgtgcctggccactttttgttagaattaatactttgaagataccatggatttggttctagaccactacaattaagcaaatatcataataaagttagtcacaagaatttattgtttccccagtgcatataaagttatatttacatggcattgtagcctattaagtatgcaatagcattctgtctaaaaagtgtgcataccttaactaaaaaatactttactatttatttatttattgagacagtcttgctctgttgcccaggctggagtgcagtggtatggtattggctcgctgtaacctccgcctctcaggttcaagcgattctcttgcctctgccttccaagtagctgggattacaggcacccgccaccacacccggctaattttatatttttagtagagaccgggtttcaccatgttggccaggctggtcttgaactcctgacctcaagtgatctgcccacctctgcctcccaaagtgctgagattacaagcgtgagccatcgcgcctggctaaaaaatacttgattgctaaaaaatgctaacaatcacctgagccttcagggagtcacgatcattttactgctgtagtcttgcctcagtgttgatggctgctgactgatagagtgatgttgctgagggttggaatggctgtgtcagtttcttaaaataacaatgaagtttgctgcattgattgactcttcctgtcatgaacgatttctctgtagcgtgtgatgctgtttgatagcattttatgcagagtagaacttctttcaaaactggaggcaatcctttcaaatcctgccgctggtttatcaattaagtgtatgcagtattctaaattgtttaactttgtctcaggaaactactttccttgctcattcagaagaaacaacaccttatccattcaagttttattatgagattgcaacagtttagtcacattgtcaaactccagttctaattctagttctcttgctatttctacgcgcctgcagtgacttccgccactgaattttttttttttttgagatggagtctggctctgtctcccaggctggagtgcagtggcacgatctcagtcagctcactgcaacttgcgcctgccgggttcaagtgattcttctgcctcagcctcctgagtagccctccactgaagtcttgaacccctcaaagtcatccacgagggttggaatcaacttcttccaaactcctgttgatgttgatattttgacctccttctgtgaaacacagatattcttaatggtatctggagtgcagttatccttctcaaaaggttttcaatttactttgcccagatccatcagaggattcactatgtatatatataaaacagctaatgtatttctaaaacaagactggaaagtagaaatgacccttgattaatgggctgcagaatgggtattgtattattaggcatgaaaacaacatgaatctccatgtacatctccatcagagctcttgggtgaccaggttcgttgtcattgagcaatgagtaatatttgaaaggaatctttcattctgagcagtaggtctcaacagtgggcttaaaatgtctagtaaagtcttgcaataaatggatgtgctgccatctaggctctgttattccatttgtagagcacagggagagtatatttagcctaattcttaagagctctacagtttttggaatggtaaatgagcactgttctacctaaagtcaacagcagcatcagcccctaacaagagagtcagcctgtcctttagtttggaaggcaggtattgacttcacctgtccagctagaagagtcatggatggcatcttccagcagggggctgtttcatctacagtgaaaatctgttgtttagtgtagccaccttcgtcagtgatcttagttagctagaccttttaggtaacttgctgcagcttctgcatcagcatttgctgctttaccttgtacttatatgttatcaagacagcttctttttttaagcccgtgaaccaacctctgctagcttccagcttttcttctgaagctttctcacctctctcagccttcatagaattgaagtgagttagggccttgctctggataaagctttggtctaaggaaatgttatggttgatttgaccttttattcagatcactcaaaactttttccatatcaacaataaggctatttcactttcttatcatttatgtgttcactggagtagcacttttaatttccttcaagaacttttcttttgcatttctagcttttgatttaaagtgagactcttcctttttgcctgaatgcttagaggccattttaggattattaattggcctaattttaatattgttttgtcttaggggatagggaggcctaaggagagggacaaagatgggggaatggctggttggtgtagtagtcagaatacacaacatttttgccgtcttccatgggtgcggtttgtggcaccccaaaacaattacagtagtaacatgaaagatcactgatcattgatcatcataatagatacaataataatgaaaaagtttgaaatactgcaagaattaccaaaatgtgatacagagacatgaagttaccacatgcttttgaaaaaattgtgctgatagacttgctcaacataggattgccacaaacttccaatttttaaaaaaatatactatttgtgaagtgcagtaaactgcagtccagtaaaatgaggtatgcctgtaaaacaaacccgcagaaaaaaaatcgtctactcagaagagcactgacaagtatcattgaattattatatctacaacttgctaatcaagctaatgtagtgtgagttgtagatacaaccattttaatgcaggggttcctgagatctgaaaattattttaagtgtgcctccagtgtagaaagattgagaaaggttgaaagtgaagatcaataatgggatgaactggaaatatgcctacctgataatacaaagcaatgagagaaacatagtatcacttccgtcatattcctgcctgcgatgcataatgtgaatccaaaattagacaaaccaaaattaagggccgttatacaaaatgaatggcttataatctttcaaagttgttaaaggaatgaaaataaagaaaggatcaaggaagtatttcagatacaaaactcaaatgggttctgaggaatagacagtctgatatgtcagtgccattttccttactttaacatttatattgtgattatgaagaagtatgtcctttttataagaaatgcatacttacgtgtttggtaggggatggtgcatcatgttggaaacccctcccctcccctcccctcccctcccctcccctccccaggcctctcgttagtagtttccaaaccttttgcatgctgaacccattgctcaaatgaaggcagaatattaaacatgtaaaggaagagcttgtgtgtgggggggggggagcggggggaaaggaggttgggggaacagagaattaggaacccctgagtgactacagaacttctgaaaaccactgttctgtaggataaaatctaaactctgaagcacattatacaaacctctatctatacacatcagtttgtctgaaattgtatatttctcaacaatattgatctatttgtatttcaatatgttgtatgctctcatatgtctgtatctttgcaaatgatattttcttctctttaacgatttttgtcttaccctgctggtaaggaagtcaccttccctctcccttctgtatatccttgtcaaggaactatggaaattgaatggcataggtcttgatacaagaacctctcttttctctttataaaaaagtcagtaaatagtggtggaacattcaggagaaagttggggacatagagactaagaaggcaatgcagtattattaggacagggggtaaactaaggcatagaggacagatttgatgaacatattatcttttttatatacattataagaagtagaaggctagaaaagtgaacatgcttgctattgcacgtctcactttccaatttcatgaagaaagcaaaaactacttctactttattacttctttttgatgttaattggtaccacatagcaagtttgcattatagtactgagctttaaaatgcaaggatatactcatgtatatacacagacaataaataataggttcttttccacattcaggaagtgaaactcagctgtccgtacgacacttactgtccatatataggcatccctcagtatctgcaggggattggttccaggaccctcacaccaaaatctaggtatactagtcctgcagaaccaacatatatgcaaagttggtcctctgtatacttgggtttctatatcccattaatgtggagaatacttttgatatgtggatatggagagctgactgtatttattgaaaaaaaatccacgtataagtgcacctgtgctgttcaaactcatgttgtttgagggacaactgtattctgttacttcctatagtttctaaaagcattaaccaacaaatacatgtaagatgcgtggaataatttttccatttcctagaaaatagtcaatcatttttttttcagattgtgaactagaaagcatagtgaatatagatttttaaacatgaaaatgtaagtgtccattttaaattgttatggatatttctgtttgctgaagttcaagactgaagactactggaaaaaatcctgtgactgagagcacatagattccttctttttaggtagagcgcaacagtcaccatgacttcagtgtttgcatatggaagctaaaatctgtctgagaaagggcaaacaatcacaggagtcattgatttatttatttgttcatttttaatgcaaattttaattgagtgaaaaagtggtggaaaaaacagttgactaaagaagatatgagaagggttaatacatgaagaagtcctcaataatattagccaccatggagatgcagattaaaaccacaatgccatactactttccatccacaagaatagctaaaattaaaagaagtcagtcaccactgaatgttggtgaaaataggaagcagctgaaactctcttacatggctggtggaagtgtaaaatggtaccattcctgtggaaaactaattgacagtttcttagaaaaaacactcaccctatgagcaagcactcctagttatttacccaggagaaatgtccacaaataggctggcacaagaatgcttatagcagctttattcagaatgaccaaaaactgaaaacaactccccaacattcatcaagagaagtgataaataaattgaggtatattcatacaatagaaagtacacagggacagaaaagaatggatttctgatacatgcgacaacacgaatatcaaaaacagtatgctgaattaaggaaaaagacaacaaaagtaatgcagcatgagtcatataaacatcatataaaaatgatgtttcaaaatccacaaaactaatctgcactgatggaacagtagttatctaaatgtgctaaggagtgattagaatgggaatgggacatgagaaaagagggaactttatggagtgatgaaaatattcaatacctttttctttttgagacagtgtctcgctctgtttcccaggctggagtgcagtgtcgcgatctcgtctcactgcaacctgtgcctcccaggttcaagtgattctcctgcctcagcctctttagtagctgggactgcaggcttgtgccgccatacccggctaattttttttttgtgtttttagtagagatgggggttcactatgttggtcaggctggtcttgaactcctgacctcaaatgatccacctgccttggccccccaaagtgctgggattgcaggcatgagccaccgcacctggctgaaatattctgtgtcttgattaaggtgttgtatatatagatatatatgtttttcaaaactcactgcgctttctactttatataaaaagtacctcaattaaattacatattaattgaaggcaaattaaaaacatctctgtctgtaactctcctactgtgagtctgttccatgttgaagaatgctcttgtcttcttttctttgctcttcttggttgggacttccctgttctaatatcaggtatgctcacgttagaaagctaggacagaggcctagaatactgatttttttccatttcaacaggcaaggtgacagttttcctagagttcacaactcttggtattccaagtcagcacatagttcacggtgaaacattctctaggaggtagagagaattgtgaccgaagaatatgataggaccaaataagtagctatactagaaggaagcacatttgagaccactaccctaaacagccaatgactacagaaccagagaaaaccagaatctgccaaatttcagaaataactcagcatctttacagggagcctctacacaatcacaatgagactctgaagagtagcaagtactgattcaaatccttttagctgtggactccactctgcctcacaatcattttagaagagggttttgagctttagaataagcccaccactgtataaaactagtgagtctgttttttaaggtaggattcccatcttagtaatcataattttggcatggcaattattaaatatgaaccacaaggagaaaaaaatgtcctcttgttattactttttaaattaggcattttaatttcatttactactgcttgatactctcttctctgggttcctgggaggtttcatttggtaagtattgttcagtaaaaattatgggacaccattgttttggactgtgctcctgccctaggccccagtggaccagatcaaactaaaatgtagtcattcatgttaactgccacataatcaaatagaaacttccaggaagcagacagatcccaaagcagaccatttttttccctgagaacaggagattccagtctagctgaatcccctgtgctttaaacccttagaaaaagtaaactgaagtaacctgatattaacaaatcagcttttttttcctgttctgtttccttgttcccaccttacaaaacccactgttgtgctgttgctcagtaggacctctcattctaccttgcagaatgggggctgccctgattcatgaaatgcaaataaatgccagttagatctgtaactaaactgttgtaattttgtcttttgacagaatgcagttaaaactcaggtatatccacactgcttttatttcgtctccttcccatttcagaaactcctgtctagatttcttttcttgctctctaaggcaaacaattaccacagttagatgaatatgcctggcaatcgctattgacagatagactctcagaaacactcgttccattttccttttcaaattcttggcaggaagactgggtggatatattgaaggaggtactgtttgattgtactgcacacagtgtggtttcaaaaatgtgtatttgaattggaaaagagaaatatatgtcaggcactggggatacaatactgaccaaaggtatataccctgaatccaaaaataaatataatgtagttgctgtaaacatattaattttaaagattgtcagaagaatatccatcttagttagacctttgcaagatatatagataagaaaatttctgaaagttacataactaaaatagaaaccagtcaaaatgaacttcattctaccctggtttcttccctctaatgttcttatctgtcaatactgtgactgaaaaagccaaacctaccaccaccaccaccactgacaaaatccaaaaaactacagatatctacaacattaattctaacaccaagtaacattataacccacttaaaactgttcttttttctttctttttttagtacagacagaacttttttttttttaatggtaagaaatatcatgattttcttataaagaccttctgtatgtacaaataaagctatactatcatagtggataaatcagtaaacaatatcttatgtaatctgtaatttttcacacaagaaatttaaaaagtttttcaggttatagaacagtatttctggacacacctaacaaggcagtagctgacattctcaaacttcaaaacaccctcactttcaatacaaataatgctgtgttgtacatttaacctaaaactaagagaaagcattgttggttggccacaacttgaatttcttattacaatgaggactgcttcaggattttaccactaaactcagccgttcagagaactaggaagatagtaaccatggtcactgttcttcaaaagcactgatttcagatttgttgaagggatatttcttagatcttcaagtttctgaaaaggtttccttcattctggttttctggatttccttgtcattctgaagttattcctcttgcacaggcaaaattagagtactcattcaataacaacaacaacaacaacaacaaagccataaaatatgccttcttttttctacaacaccaatttagctactcaagatacagaactaaaatattagcagaaaatcttgtaggtatgaagccagttatgtattcacattagtaaagatgattccactgcattcatttaatcagcaaacatttacagaatgcctactacataccaacaatatattagtgactgcatattcatttaatcccgaactctgaaatcattattcctggtttacaaaataggaaacaggcttggattaaggttgcttgcccaaagatttatagttagtaagattcactaccaagtttgaaactcagatatgtctgagccaaaatttctgctccttccactaagccaagctgtcttccagcatggcttccagcatacttagtatcttgctgtatcaagagaaaacaaggtacaggtgacagtgacgtgatgccattatgactatctctttttatataaaaagacccttgttgagataactacaactctctctttctcagacctcctacacattgcttttccttcaatcatcagggtcatgagccttctcccctctcctcccccgccgccccccaccacccaacttccccctaacaaagtaaaagaaatcaaatgagatttgattaaagtgttttgtctagactgcttcaggactaaagggtcttggtaatttgtaccagcacctcacttcttccccacgcccaaaaactcacgtacacagtttgattgttcttgctttctaaagtgttctcttttttttgagatggagtttcgctcttgttgcccatgctggagtgcaatgacccgatctcggctcaacacaacctccgcctcccaggttcaagtgattctcctgcctcggcctcccaagtagctgggattataggcatgtgtcaccatgcccagctaatttttgtatttttagtagagacggagtttctccatgttggttaggctggtctcaaactccctacctcaggtgatccacccgccttggcctcccaaagtgctgggattacaggcatgagcccggccaaagtgttctgaaagctatgtgtgaatctgttaagtacaatctatacttacatttgattataaatattttgacgatctgaattggtaagattttaggcaaaacaacaaaatcaaatcccgtggactctgacccaaagaatatattcagctttgtttgaatatatttcatcttgcttccttaccaattctcaacacaactccagaataactgttattaactcttattgaatcttattttgtactaagccttgttaaatgttttacctatgaattgtgatttcattgttacagcaaacctatgatatagatgctatataacagatgaagaaatgaggttcagaacctgtgctacgctgcctcgcaggcacaatccatctgataaaagtagtcccttgaatctctctttctgaattccagtcccaggacagtggaaatacacagtattgtggtcaaagataaaccattcttggctccaggtgagctaatggttttagataagaataaagaatatttattagaaataaaaaattttgtaagtataaaattagactaggaaaaagctcccggttgaattttatatttataaaatcctttactgaagttgaaatcttctccttgaaatttctgcttggtatggcctctctgtttgcctcacaagtgaaatttaatcctaatgttaccttattttccaagcataaccacaccagtaggctgctttgtcatgagtttagtatggtgtcagtagaaacgagaccagcagtcattagggttacctaattcaaatcttgactcattttgggtacttcctacaagattagaataattatcttccaaaccaaaaacatacccaaggttccatgggaaagggtgtagcttcaactctttttaggtggcaagaaaatcattctctaacctctcaaaggtcaggaatagggtcgatggtccttaaaatttggtctggggaccactggttgctgaaccttttgcaggaggtctgaaaggtcagacctgttttcacaatacatgttaagaagttaatggcttttttgttgtcattcttttccaagtgtatttgattatacaacttgggatgatgttcctctgatagttaatgcaattatacttatgttttaaaagtttgttagttttgatttctaatacagtaagtctcaacagatagaactcacataacaaaacacttttgggagtccttcataatttttaagagtgtaaaggaggttctaagaccaaaaggtgtggaaactgctcttctaggtttcagaattatgaagcatacaaagactcttcatctggaagggtttagaggtaattttatctaatccccttattttacaggtttagaaactgattctagacatttaagttcccagactaatgtcacagaagctaatgaattgcagaggttaattggaagcctggtcttaacactcccaggttatcttaatgagttcatgaggatggcatatggataatgcacttcaaagggtgttgtaagtattaactaagttaatacaggtcaaatgcatatattagcactcaatgcacggccattgatcaataaatgctagtggttctgatcagtgagaatctaacctctgcttaaatacctttagtcatcagcagcttccactccctgagtaacatgttgcatttcttgatcaattatatttttacagaattcttcctttactgaagttgaaatcgtctccttgaaatttctacttggtatggcctctctgtttgctacacaaataaatttaatcctaattttatctagcttattttccaagcataaccacaccaatttcattaaatgattcctcatgtggcatgactttaaactccgtcaccatcctatttgtttttctcaaagagctccagttgactgctcctgtgaaattgtccatctattaatgtaaatgttttttctaattttacagagctccccgttgtattgtgtacagtgttaaaatagttttctgagatttcttgactctgttttcccaagtttcttgtggcccttctctttccttcgtctctattctgtgcggtttttatttcactcccacagtttctcattgctgtgaggccctgttatggaatgagagccctggttttgaaagttcacagaggctagacttctcttgtccctgtagtcctggctgagggcccactacacttgtctgttatccgagtgggcaaacgacctacccgttttcatctgctgggcggccggttatttggggggatccccctgttacaggtctgatctctgttgcttcctttgggaggccgaggcgggcggatcaccaggtcaggagtttgagaccagcctgaccaatatggtgacactcctgtctctactaaaaatgcaaaaactagctgggcatggtgacgtgcgcctgtagtcccagctactctggaggctgaggcagaagaatcgcttgaacccgggaggcggaggctacagtgagtcgagattgtgccactgcactccagcctgggcaacagagcgagactgtttaaaaaaaaaaaaaaaaagtttgtagccattatctctggaaatatttactcttcctcattcttctgcttatctctttctggaactccaactagatatatactagacctttgattctatttttccacacctcttaacctgtctagcttatttagtcatacatctctcaagctgcattcttccttggagctttatctgtaggaattctttgagccttgattgagtttatattgcttcagagaaaactaaggtttgcttcagctagttgcccaggaacattaccacctggttaccacttttaattaaggtcactgcttgaggatttcagagcgacacagagccctgtatgagggcctgtttatggttataaattcttggggtgtaggcaggggtggggatcctgcttctttacctggagctaaaactgagacagaaaaatccctgactgtccatttttgtgtggtgggtttattttctgttcaccctgaacaatgataggtgttcaccttgtagagctccccgctttatgtgggggtttcctattagagaactatcatatgtggcctgttggcttattttcttgccttcagcacctgtgccagtacataagttagaaacccaaggtttccaggtttcgaaaaactctcagggcaaaagttcgttttagcctatgcttagctcccagggtcctttgtacttggccatatggatttctttttttttttttcttcatgtcaacactgtggttatatttatctgtctaacctactcttttaatttttgttttatctggtattttaattgtttcatttgagaaagtttttcatagtatctgtttggtagttggccattctactaggagtttaggagttatacttaactccttccagggagatgttggaagatttttactaaaaatacaatatttaaggtgggtattgaagtactatcagaggggacctggggtggagtatgaaaacaaaacaaaaccttacaaacgggaataattaagagttaggatatgtgagatgtttggttttgctgggcttaaaatagaattgtggggtatggaattgctgcaaatgaggaagatggactcagagatgaggctcaagagaggccacatgcaacttttgagagtctttgtgtgtcacagtaaggaagatgaacttgtgaaatcaccaaagggtggaatatataaggaggaagctgacactgtcatatctatgccttaggatgtttattttggcagcagtgaaaacaaatcaggtagacaagagtggagcattgctcttcaaaatttagtcattgactggcagtaatggcatcatctgggagcttgttagaaatgcagaatctcgggtcctatttcagatttaccaactcagaatctgcattttaacaagactcctaagtgtttcatatgcatagtcagttgatgtctcaaccagtgacctgcagagccagtgatctgcaaagcaagtgaacgttagctttattttaaatttcaagaaagaagtcttaatttgcctagagtacatatcatttgatgttcacagtgtcactttatttgcctaataactagctgactctagatccttagcagcattagatttagtatttgaggttttgaccctatgtacctttgataagtagtgatttgtaacttatgaattaaatttgaattccttaacatgttgctagttacaaaactctagtgtctctagcagactattaagaaattgagcaggtttcgttctccattcactgttaacacatgcggtaactcaccaggcgcttaaaacaagtgggctgtggtgcagggtacttcttgtttagtgacagaaatgaaaagatctaagaatatgatggttttaaataaatatgataagagatgaagagagttttaagtaatagaactattctaagttttggatgtttggtttagtgtctctagctatatttctgtttaatgtcaaggcataatatattcgaaccattttatttattaaatttaataaacattgattgtcctattagtcaaagtttcagaaaaatgcaaaaagtcttgttctcaaaggaatgctccctggaccatgcacatcaaagtcgtgggtggctgcttgtgggggtagaaaatattaaaaatgcagaaactgggccctactgccgaatcccaatgtacattttaaaataagcagcttcctggccaggtacggtggctttcacctgtaatcccagtattttgggaggctgaggcaggaggatcacttgaactcaggagttcaagcctgggcaacatagtgggacccccatctctgcaaaaaatggaaaaaaagtaaaagcatctcccaaggaattctgccagcaggaaagttgtgttttcccccctcaaatctggaaaccataattgttcactttttgaccttttactggaatacagcatactctgagaaaagtaacaacactcaaataaaaaaatagaacattctattccagaacctcctctagtgactccttctagaaagcagtctagcaccccacccctccaaacacaaacataaccaccatagtgacttttaacaccatagattagtttttccttttttgaactctttaaagtggaataatacaatttatactctgtctgttttgtgttgtttttgcttagcattatgtctgtaaaatttgtctatattgttagctgcagtttgtcattctcattctcattgctgtgtggttctctgttgtttaaaagtaccagtggtaaaattatcatttatgtggtttatctctgatggacattagaggtatggtggtaccactgataggcaccaaaatcaagtttaataaccactgttgtatattatttgggaaaatgtgtactcttgacatgtttggcaaatttttatttctccaatctaaaatttagaaaattataattttaaaattatcaataaaaatttacaaagtttttactgtcaaatattatctaatagctcaactagctcatgctagagtaatacagccatgtaatacagcattaccaacttttctaagtggtctatagcactgaggaattaaatagcaaataagggaagcatttcttcatgaaatcatttcttttaataaattaaaaagaaatgagagtattagaataccaccattttgccaccttcagtgtattaatggatggaggcaatgaatatcaacagctgctaaaatcataagaaggaaaccagatgctagatgacacataatgaagtaacacattattagacaaaggaacaaaccaagttcaataaagcctctggatccagcttccaatttgccacaaataaagagaccagatgaatatgctgaattgcattatgtgtaaataatcagtcaaatctacactacgaaaagtcagatcaaacataaattttaagaaaaagaaaagaatggaaaataaacctgtagattaaaagagactgaatagaagtagcaactcttcttaaaaatggtcaagattaaataatagttatctagggaggcttacttagctgataaagtgataaatacaggatgtaattaagaataatttaaaagaagtgagttacttagaggaagggaaggggctatgactgaatcagcacttggaggagcttctgggctcgctggcaaattgctgtgtggtggtcacaagaatgtattctcttaatatgctaaggtataaagtttttgtatagttttctgtatctgtattttattttactctaaaggaagtagttttttaaaaaagattatagatttgctaatctaatataaactcccctagagcttcatcagtaatagtctagtgtcatctggattatcttcagcaatcattttcattctaaattgtcatagtgtcatctcaaagcagaaagagacagagagtttgacaaagtgtcttaaaatgcctgatgtctgtcttaatgattctaatagaaactcttcagtacaatactcagacttactgcgcttacaactacataatggcttataaatttgggaaactcaacagatttgggaatacaacacatatcttgaagccagttaatttactttttacatacctcttcactattccactaccagtgtgcaactggtaattcagttgaattcataaagaattcactgagtttttctgaatttcttctgatttcaagaggctagaagaactcagattataaagcatcaggttatcacttttactatataggcacaccatggtttattgcactttgcttctgattttttttttaaacaaattgaagggttggagcaatcctgtgttgagcaagtctcttggtgccattttccagcagctcactgtgtgtctctgtgtcccattttggtaattctggcaatatttcaatctttttcattattattatacctattatggttatctatgatcagcgatctcttttatgttactatcataattgtttggggatgccatgaaccacacccatagaagaataaaagatggcaaacttaataaatgttgtatgtattctgaccactccaccaaccagctgttcccatctctcttttctcaggcctttttattccctgagacacaacattgaaattttgccaattaataaccctacagtggcttctaagtgttcaagtgaaaagaagagttgcatgtctctcattttaaatcaaaagctagaaatgattagtgaagaaggcatgttgaaagcagagacagggcaaaagctaggccttttgtgccaaacatccaagttgtgagtacagaggaaaagttcctttctttttttcactttttcgtatgtttaaaaagtagagacagggtctcgctatgttgatcaggctgttcttgaactcctgacctcaagcagtcctcccacctcggcttcctcaagtgctgggattataagcatgagccactacacccagctgaaaagttcttgaaggaaattaaaagtgctactctggtgaacacatgaattataagcaaaacagccttattgctgatatggagaaagttttagtgtctggatagaagatcaaatcaaccataacattcccttaaacaaaagcctaatccagagcaaggcccgaacttacttcaattctatgaagggtaagaggggaggaagcttcagaagaaaagttggaagctagcagtttggttcctgaggtttaaggaaataagctgtctcgataacatgtaagtacaaggtaaagtagcaagtgctgatggagaagctgctgcagcatgttatctagaatgtctagctaagatcactgatgaaggtggctaccctaaaagattttcaatgtagatgaaacagcactctattggaagatgccatctaagacttttctagctggataggggaagtcagtacctggcttcaaaacatcaaaggacaggctgactctcttgttaggggctaatgctgctggtgacctcaagtggaagccagtgctcattggtcattccgaaaatcacagggtcctaagaattatgctaaatctactctgcccatgctctgtaaatggaacagagcctggatgacagcacagtttgctagatatgttaagcccactcttgagtcctactgctctcagtgaaagattcctttcaaaatattactgctcactgacaatgcacctggtaacccaagaactctgatggagatgtacaaggagattcctattttttcatgcttgataaacataataacatctattgtgtagcccgtggatcaaggagtcatttctactttcaagttttattatttaaaaaatatatttcttaaggctgtagctgccgcagtgattcctgtgatgaatctgggcaaagtaaaccaaaaaccttctgggaaggattcaccattctaagtaccattgagaacattcgtgatttatgggagggggtcaaaatatcagcattaataagagttgggaagaaattgattctacccccatgggcaactttgaagggctcaagactacagtggaggaagtcactgcagttgtggtagaaatagcaagagaagtagaagtagaacttgacacagcgtgacaattgctgaaatctcaagataaaatttgaatggctgaggtgttgctttttattgatgagcaaagaaagctgtttcttgagatggaacctactcctagtgaagaggctttgaaaattgttgaaatatcaacaaaggacttagaatattacataaaattagttgacaaattgataaagcagcggtggtttgggaggattgcctccaatcttgaaagaagatctacagttaggtaaaatgctgtcacatagcctagtgtctttcatgaaaggaagagtcaattgatgtggctaactttattgttgtcttattttaagaaattgccacagccatactgattagtcagcagccatcaatatcaagataagaccccccaccggcaaaaaaattggactcactgaagtctcagttgatcattagcatttttttaagcagtatagtccttttaaattaaggtatgtacattttttttacacataatgctattacacacttaatagtagtgtaaatataacttttattgcactgggaaaccaaaacattttttgtgacctgctgtattgcaatattacctttattgcagtggtctggaattgaacctgcagttttctgaggtgtaagtattggtgaaatcattaacctcctcctctgtgtgtgtggtttcttcaactcacaaaggatagcagccccagtgaaagtcgttacagaaggcagataaactccattttttttaagactttgccactctgtgtgtgtgtgtgtgtgtgtgtgtgtgtgtgtgtgtgtgtgtttaccttatcctagtgggccttaccacacatttctattatgtgagatccaaaagtgatgtggtatacacaagagtaattttcaccccattcttaaaactgaaaatgatgtttaaatcactttttcttgggggaaaattcaaccccgtggtaattaagcttcacttttcctgaaattaatctttttataaattttataaacttataagaaatgtaatacattttgcttaagtaactagcataagccaaaatggcacttcatttttcttaggctcagcagatttaatttaataaagattataaattgattttaattaatgatgtttacgaaatgaaaattaattgacagtgttgaatagtaaagctgctaaaaccataagccaaagcaatatgaataaaagtataatttagacacaattttaaaccagattttgaaaaactttactcggtgatatggtcaggctcaattgtatgcctgctagttagattacttcttgtataggctgatatatgcataaaattattatttttgaattttaaataaaattatatttatctctttaatgtgaatttacctctttaatgtaaaaattatatttgttttttgtccttgtttcttactgcacatatcaattccaggtcaagcatgagataagcaaatcatgttaatttcattttcaactgaaataagactatttctgagcttattcttgtttgctgaataaaaaaagattgttcatatgtgcgagaaattgctgcagcataatgttcactgtttttctgtgagtagcaggataatcttttcttcatagaaatctacatcttgtctgggaaagattagtaaaactcatctttaatgtatgataaaactgcagatctttttccttttttctcaagtcaaattttcacagtcagaacattcagaaacaggatcccttttccagttctacacttgtgttcaagtgaaggaaaatctgttcagttttttttctgcagctcctccaggtgatttccagtaagacttgagacttgctgatatccttcctcactctcaagcccaaacagcaatagaaacatttcaagattttcttttgtaacatgtttttcaaaagctcattttccttttacatccaagaatgttgtcctttgaaataaagaaaacccaaccattttcttcacaccttacagagactgaaaaataagtactacgtaggctagtttctacagccattaatgtttaagtattcaacagactgtagcctactgttttctttaaaggacccatttcagttcaaataccctattgagaagttttccactgctaagtggattttgtgtgtgtgtgtgtgtgtgtgtgtgtgtgtgtgtggtaagagctgttctttaaatgagtgaaatgacctttgtttaatgaagttaaccattttataacatctttcagatgttaaaacattttgccccaagagcttttgatatcagtactcttaacacagatgttttttgtgttagtttgggtcttctgagacacagatgtcaagacaagatttgatgcgcagggaatctcccaccccaccctactaccctcctattgtcctttggagcaatccccattctagtacttctgccctgcttggtagcttgctgggagaagcccagaggcagcaaggccaggggtggttgccatggattccaaggtgcgatagatggaggctgtcaagcagttctgttcctcatagcaggttaggttgaggggatatctgagtagggtaccactgtggccactgcaccctcctcttcagcctttgacatctttccctcatgtggacactctttactgtgttacgcacccacagggatgttgtcactgtgttctgcctttgacctacgggggcttctttactatatggattattcctcatgcttcttagagtcaagctttgccaccttgcccccttgttggtctgcctctgttcctccccgccgccatccctcactacagaaaggctcttttcattctgctttgactcccaaattttggactacctgcctgccacatacatacctaacttgcttggctccatctaatagctttttgactaaatttttgaggaaaagaaggaagaagagccatctgggtttcttacatctgcaactagctagaatatgattccattcactgaaatagagaaaataataggaggctctaagaacaaatttgggccttacgtatgtgtgcatgttgtggggaaatagaagtttggatgttaaaataatgaatttggtgtgactttgggacaccttcttgaaattaataggctcagtagaggagtctgactggagataatagtatggggagtcattagcttctgtgtgatagttggaaccctgactttcaacgaaacaacaaaggagggaggagctagcgatggagcacagtaacagtgctgcctgagggatgcactgaggaatgtaccaaggaaaattaagggacaggagagagttgtaaagagagctagtgaccaacagaatataaagatacaaaaatggcaaaagagtctttgagatttaacaaccagtttaaaatttagttattatggagtaagcccatatcacacaggtggtggcgtatcacacagggattaaatttagccaaaacaaaatatgtattataattcaaataacaaaaaatatatattgtcatgtggactgaggaatagtcttttgcatcctttccagtaaagatatatatgattgactagtgaagtctatttaaattattcagtgtacatccataaaactttatcaattactttctgtgtatatgatgacacttgccagtattgcccattttgtgctgattttgttagtgtacattactaaggagcttttcatcaaattttgcagtccctgaaagattttcatctttaaagttacaaatgtgatttctcagctgcagtatagaatatatggaaccagaaatactcaaaaaataattgttttcgaagtattaatctttttagtcacagttgtttttttacatcctgtgctgaaaataacaagaaatttgatacagagggaaaaatgatttattatgacttagtagacaatttacaaatgtgtgttaagatattaggatatatgtcctaccagtttcaaaagtactacaagtgacttgttcaatacagagtacaactttaaaaaatgtatttaaagtaattgacgttgtgtttgtgacctggctcgaagttcttttttggtgaagagcatgcttagtacatgattgtctttaaaaagatctgataattatttactcagtaaatgttttgagtgccttatgagtcaggcatttttgtgggtgctggagataatagtgatgaaaaacaaaagtcccttttccttatagaacttaaattctagtgtgggaaggcagatagtacagaaataaattgatggatggatagatggataggtaggtatttgctatatagcaggtactatttttgcttttatatagtgctgtggaaatgagtaaagtcaggacaaaggaaaagagaaggtgatgctggggggtattattttaagttggatggttagggaaagtatcattgaataggggacatttgaacagagtcctctatgaaggaagtaaaagaaataaaaagaggaatagctagcacaaagactctgaggttgcagcacactttacccctcaagaaagaacggtgacagaaagggtggaacaaagtgagagagtagtaaaatatgagttcacagtggtggggatgtatgtagatgatagaaggacccaacaggcaaccataaaagacattggcttttactctgagtgaaatgggaagctcttagtgggtgttgagcagtggagtaataagataaaacttatttcatcatgcatttcaggtacttactcctaatcatagtaattaataaattattaatttggggtatagaaagttcatatatgaagtggagggtgttggctcttttaagaattcagtgaaaatcctaaacttcttgcagaaagtgattccaagctttgagttattcttcctgatgatcagtacagttggtttactttcttgttatctttgtcctaaagcttcttaaatcactttgtagctcaagcctaatggattatacctgcccatgtaaattctgaaaatgttaatgttgcctagtgattcagaggctttagtaatttacttaaactacttcttgttttattggtataaactgtattcctcagtgtctactatgatttcaaagttagtatttgccttggaatttttctttgaagctggcaactctagttcaatataagacaggctctcagagctccacttatttaacaactgtatctatgcccacttttattcctctaagcattcctagaataagcatttcaaatggttttgaattatcaaaggtctttttgaaaaacaaggttattgagaaaatgtttaaaaagttcatgagaaagttgtctaaaatacacccccctcccccaaggtaggcctgaaatgccactaaatcaacaaaggatagtcactaaaagttaccctgtattttctaggacttggggaaagtcatggagtagctgtgctttctctaagtaacctattttaaatttttttgaagagcaaaattattatacctctttttcatccagaatggagctgactgtaggcatctttttaaagtacccataggtcaggacctctctggactttccactaccttgaaagacactgccagaagaatgttgttccccacacttaaaaaaggaaaagtaatgttcttttctccagccattattttatgcaaagtccaactttattttatctgagctatctgaactttcaatttatttgaaacatttattgattaatatctataatggagcttttaatttctctgatcatttatcctttgttaggttagcagaactgtaacaacacagtcactttcacagccacgaatgatacttttatagtcatttgtggacatatactgtgcagagtatcacaaagtttgagccacctgacaaacttatttccagttgagatctgcagggtgatgctctgccttcttgttgcagctctcataccatgaacaagtgtcattttcatggtccatgaggaaaaagcattttcctcattttggtgctttttgttagtgattgtgcagtttagaatggcccccaaacatagcctgaagttctgtttaatgttccgaagtgcaggaaggctgtaatttgccttaaagataaactaatgtgtgttaaagaaacttaattcaggcattagttataatgctgttgaccatgagttcgatgctaatgaatcaatgtatattaaagatatatttaggcagaaacacgcataaaaaaggttatgcattgatcagttggcaacagtgttgtgaccagaggcttgtgagaactgtatttcccctaggagcaatggctcagtatttgttaattcagtggttgcagcaattttatagaacacaattactgtgaatgggaatcaactgtatttgattaacggtggtgatttatagggactttagataccagaaatgtttcataattccctttctctgaaatcactgttttaatatgtttaaatgcatgcatgcagagttgtgatgttaaacataattttactgtgggttctggtcaaaaaagatgaaatgtcattggttaacttgaaagagacattattctaaacattatcctccagaaaattgacatgtacaggaagcatattgaatgctcagcaaataatttgttttagagtaataatctttgagtattgtagtgattcgagttttggaaaagaaggcagtatcagtgttagagaataatattctttcaggattttatgtagttactttaaggtgcatgaaaggagactcagttgggtgttaaattcttgtccctgctttacttgaaactagtaatcttgagaaatttactaaatcattttgagccttgattaccttgcctgcaaagtgaggaacattttcaatttaaaattctatttcttttattagtattcttcctgaccttgaatcatttctattcccatcatgtccagttgccaagaaaaccatgcaacttaatgttgtttgttagccatcagattttattttactgaactcaagttcagtcacatcagttaccgataaaataataagttctatattaatatttgatatatcttgacattttgtattatggtaggaagaaataaaagaccttcctcaaattttaggatatgggcttctgtttgttgatgtttgtgttttatgatacactgttgtaaatcatactaaaggttttctctgaaaaagactagaattgacaatacttcatttgttagcagtttcaagttttagatcacgggtgcataatttcttgtgtgtgcacaacatgttggcattttatctgacttcaaagatgtccatatagataccagcaaaggataaaatgtaagaatgaatatcatgaaaagatgctgtatcagataaaattctagagcctaggttaaaaaacataaaggcaaacatgcttgatatataaaaattgagaaatatgataaaaagaagtaagtttaaagcatcagtaataccactgcctaagatgcagtttattttgaaatgttgtcttctagtcttcatacagtttaaaaatcatactataatcacaatttccagcattttccccttagcataatatattataacatccatgtttttaaaaatattttatgaacgtcatgtttagggattacaccatatatatcccatctcatagattcctttatattgaacatttggatttttatttacatttttatttacatttatttttatctttattttttgctttcgtggataaactgcagtgagcatcctctgtataaattttttttttctgttttaggattacttccttaggatagattgccagaagtggagttactgggtcagagggtatgaacttatgaactttttttttaaataaattttttgttcattttctgtccagtcatttgtaaaaaaattaaaataataatgattataattgttacctgctagaaaactgtgtctgaaggcaagattctgtgatcagaaaagtttgggaaatacccagggtaaaaagccttttaatctgatttacctcagcatttcccaaattaactgaacactgaaaattttttttgatacacttcttaaaattttgtggaagttttatataggatatagtctatgaactactgatgtaaaattaaaattgttttatttgcttgaaatattatgttttattggtcaaaggaattaaactataaatcttcatgctaaaaattattaaaagggattagtgttgtttactatggtttttgtgcatgtctttataaagtcttataacttttaaaattgaaatgttctatattgtttactaaagaacattttaatgccttggtggcatcaatacttttttgcaatcattaatgatatttagaaagtagacatataacatgaaagtagaacataatatagattgtacaaatcttgttttttaccctattttcccctgcag

SEQ ID NO: 5 - RNA, 23 nt, Homo sapiens
uuauugcuuaagaauacgcguag

SEQ ID NO: 6 - RNA, 102 nt, Homo sapiens
gguccucugacucucuucggugacggguauucuuggguggauaauacggauuacguuguuauugcuuaagaauacgcguagucgaggagaguaccagcggca

SEQ ID NO: 7 - DNA, 2469 bp, Homo sapiens
agatggtgtagatcagatcgatttgattgcattagatgattttttcccttccccactcctttctggaagctcgcatcagctgaaggctatcgcctgggactcctcggaagcatgagcaagccgccaccacgcgaaggcactggggcacagccagcgcgaggcgccgaggtcccttcccaaggcttgttaacactgtaacccggcactcggagagaagaagcagctcacactgcccagagcctacctcactgcacatcagatgactccctggcttctacacacagttggagttccgcttgaaacctggatttagaggggttctctggccgccatggcactcaatcataccacctagagtggactggccgagaccagactgggtaccaagcagagaagtgcagaggaaagcactgggagagcaccagaattggaaatagagcggccatttggatttgggcaggaagcagccgagcacagctttggatccttctttagggaaatcgagttatggatttatggtcccggtcaagctcagcccatccccaggcaggggcgggctcagcgagcagcaagagttctggtggcggcggcggcggcagtagcagcggcagcggtagcagcggcagcggtagcagcggcagcggcagcttggtcctctgactctcttcggtgacgggtattcttgggtggataatacggattacgttgttattgcttaagaatacgcgtagtcgaggagagtaccagcggcaggggggcagcggccgccctccccagcccaccagctggccactaaacgcccgtggttgccaaggcatccaaagcctctgggatgtgttctgactgtaaaaactctgatgttgtgaaaaaagcttacgctttgcctccactcaaaccagatggtgtttcgctcttattgcccaggctggagtgcaatgacgtgatcttgactcaccacagcctctgcatccaggattcaagctattcccctgcctcagcctcccaaaatgctgggattataggcgtgagccaccacgcctggccagcattcccaatttttaaaaatgaatgattggcacaaatcttagaaagccattttctgtagatttgaaagcaatgctatttacattgttactactttcttgttaaatcttgcatgtctgcagtatgtgttgtaatagaaacctaagattatgatctgctgtattcatatttgaagaagaaaatttcagactgtataatcaactagttgatgattcatatttgcttgtacaaagttaaaagtgtaacttgccagaaaagaaggaagcctgaaaagtattctaaatacattaataagaagggttctacatgaattaatttttgttttgccatctacagagttcctgccacattctaggcacttcatatttgctgcaacatttattcagacattgacagaacaagagaaacgaagttaaattttaagtaccatggattgaaattaaatttagggaagatattttatagtatgaattgttcatctgtatttaacaaggtattcatttattttgggcgatttaaggaaggtcctttctggaaacaggattacaaacatatggacctatttagtcaatttcaaccttgtgattttgaatctgacaggttctcagctgcttttattaaataacggattttcttaataattactgtactcaaacttagcaaaaagctctatttatagcccagttttttagtcacacactattgtgtcttgtcaaattgaaaccatatactacattctttacttattaagatggtctttctttgtaataattttggagtaaatagtttacttatctaaacctctgatttctgatttaacagatttttgaagcatttattttccttaccatacataaaaattgtcagttgaggacaaggaaggattaacctggactacggtgaataattgttcaggttgcttactgtgtaactccagaggagcattcacatggtacaatttgcagatttaagtatttattacaaccattttctggcagataacagtggaacaccctgttctgttaaaattagtttattatgacaaattgcctacagatggacataaactgtcttgaggaagggcacctgctttggactgaatcgtgtccccccaaaatcaaatgttgaagcctaatctctaatatgatggtatttggagatggggcctttgggagataactaggtttagatgaggtcaagagtgtggggccttcctgattagtaccctgaaaagagaaaacaccagagagcttgccctctctccctcttaccccacaggcacacaaagaggtcatgtgagtacacagtgagataacaaccacctatgagaaaacagaagaggcttcagagtgaaatctactttgctggtactgtaatcttggacattattctctagaactgtgagataataaatttatcttattt

SEQ ID NO: 8 - RNA, 21 nt, Homo sapiens
agaccuggcccagaccucagc

SEQ ID NO: 9 - RNA, 75 nt, Homo sapiens
guggggagccugguuagaccuggcccagaccucagcuacacaagcugauggacugagucaggggccacacucucc

SEQ ID NO: 10 - DNA, 1037 bp, Homo sapiens
ctgtgggacagaggaacaggcagagatcagagggcaggctcaggttgggaggagtggggagcctggttagacctggcccagacctcagctacacaagctgatggactgagtcaggggccacactctccctcctctggtgatgtgacctcagctggtttcttcccactcggccatgggtttcccatcctggagtgggattaagaatccttgtcctggccctgtgcagtggccacacctgtaatcccgacactttgggaagcttagatgggagaatccctaggggccaggagttcaataccagcctgggcaacatagggagaccctgtctctacaaaaaaaatttttaacaattagcccggtgtggtggtgtgagcctgtagtcctagctacttagaggcagatgtgggaggatcacttgagcccagtttgaggctagtccaggcaacatggcaagatcctatctctaccaaaaatatatataaacgtgcgtgtgtgtgtgtgtgtgtgtgtgtgtataaatatataaaagaatccttgtcctgcctgtctcatgggcagcttggaggaaacactgtttttttgttttttttttttttgagatggagttttgctcttgttgcccaggctggagtgcaatggcacgatctcagctcaactgcaacctccacctcctgggtttaagcgattttcctgcctcatcctcccgagtagctgagattacaggtgcccaccaccacacctggctaattttttgcatttttagtagagatggggtttcaccatgttggccaggatggtctcgaactcctgacctcaggtgagccaccccactcggcctcccgaagtgctgggattacaggcatgagccactgcgcccagcctggaaacactattgacaagtgaggaggcctagtccattgagtatcagctagggctacaaacttccaaatcggtgaatcaggtccagagagggacaagtgccccagggttacacaatcatttgctgaagcagaggttgctgccatctttggcctcac

SEQ ID NO: 11 - RNA, 23 nt, Homo sapiens
ggcagguucucacccucucuagg

SEQ ID NO: 12 - RNA, 98 nt, Homo sapiens
guguaguagagcuaggaggagaggguccuggagaagcguggaccgguccggguggguuccggcagguucucacccucucuaggccccauucuccucug

SEQ ID NO: 13 - DNA, 1412 bp, Homo sapiens
gtgagggcgggcgcgggccagcggccgggaagccctaggccaggcccctcccctgaaggaagggcatagggcgggtcctgcctcagggggcttgcgaggaccggccaggttcatctcatgcagcatcagacaaccactatgcagagggattttatgacgtttttgaaaaattgggaagacaatggtttgacacccactttgcaggtttagacgaagagatgcgtactgtcaagctggcctgttctctgtccccgaggcagtcagccagcaccctgcagccccgcgccaaccccacactctgctaagccctcgctttggggcttgagggagacagaccctgcttcgaaggaccctggagggagggttctgtcctgcttgggccaggatgcccagcccctggggaccccggggggacatgctggaagaagtggcgaaggacacgtggccccgtcagccccagacgccgcacggctgtcctctccaacaatatcctggtgctgagtgatgactcaggcgactccagcatcagtgattttgttgaagagggcagctgccagcctcccgacctgcctgccgggccccagctgccctgcccccaaccccaacccaccccactccaccccctaggcccaggacacatggccctgtagcgatcccctggcacgcagacatgggttttatgtggggagggacaggctgggttggcctctgtccccaccctgagtcctgagcacagaagtaatacggcagctgtggtaatatctacccagtaccctgtgcctcctcacacccacgtgaccagccaggcagggttcaaagccagcagccaaggcaggctgggttggaggtagtgccaggcgtaacctgcattctttccagaccctacccaaccctggggccagtggtggctcaagtgagagtgagctccagctctgagtgggcatggcagggctggaccctaaaactggactccggcagccggcaggacccctgggacactccaggcctcagtttccccatcaattcccacctcctggggagccgagagtgatagtgtagtagagctaggaggagagggtcctggagaagcgtggaccggtccgggtgggttccggcaggttctcaccctctctaggccccattctcctctgcactgtaacatttgaggcccacgcacacagtccctccccaggtctcagggttgggcacagagtagggccctgggcagggatggggggtggcagtgtctccaacgccccttccagcctggactgtgagccatccaagtgttggcaaaggaccctgtgctggatgcccccgcccggcacaccccactgaccctccccctgcccccacccggcacaccctgctcaccctgctcaccctgcccctgcccctgcccctgcctgcag

SEQ ID NO: 14 - protein, 6 aa, Artificial Sequence
  synthetic peptide
GGGGDD

SEQ ID NO: 15 - protein, 8 aa, Artificial Sequence
  synthetic peptide
GGGGGGDD

SEQ ID NO: 16 - protein, 10 aa, Artificial Sequence
  synthetic peptide
GGGGGGGGDD

SEQ ID NO: 17 - protein, 12 aa, Artificial Sequence
  synthetic peptide
GGGGGGGGGGDD

SEQ ID NO: 18 - protein, 7 aa, Artificial Sequence
  synthetic peptide
AAAAAAD

SEQ ID NO: 19 - protein, 8 aa, Artificial Sequence
  synthetic peptide
AAAAAADD

SEQ ID NO: 20 - protein, 7 aa, Artificial Sequence
  synthetic peptide
AAAAAAK

SEQ ID NO: 21 - protein, 8 aa, Artificial Sequence
  synthetic peptide
AAAAAAKK

SEQ ID NO: 22 - protein, 7 aa, Artificial Sequence
  synthetic peptide
VVVVVVD

SEQ ID NO: 23 - protein, 8 aa, Artificial Sequence
  synthetic peptide
VVVVVVDD

SEQ ID NO: 24 - protein, 7 aa, Artificial Sequence
  synthetic peptide
VVVVVVK

SEQ ID NO: 25 - protein, 8 aa, Artificial Sequence
  synthetic peptide
VVVVVVKK

SEQ ID NO: 26 - protein, 7 aa, Artificial Sequence
  synthetic peptide
LLLLLLD

SEQ ID NO: 27 - protein, 8 aa, Artificial Sequence
  synthetic peptide
LLLLLLDD

SEQ ID NO: 28 - protein, 7 aa, Artificial Sequence
  synthetic peptide
LLLLLLK

SEQ ID NO: 29 - protein, 8 aa, Artificial Sequence
  synthetic peptide
LLLLLLKK

SEQ ID NO: 30 - RNA, 19 nt, Artificial Sequence
  synthetic RNA
uucuccgaacgugucacgu

SEQ ID NO: 31 - RNA, 19 nt, Artificial Sequence
  synthetic RNA
acgucacacguucggagaa

SEQ ID NO: 32 - RNA, 22 nt, Artificial Sequence
  synthetic RNA
uaccugaauucccaaaagcuuu